European Patent Specification EP 3 299 476 B1, published July 19, 2023. Title: COMPOSITIONS FOR RNA-CHROMATIN INTERACTION ANALYSIS AND USES THEREOF. Applicant: THE JACKSON LABORATORY. The sequence listing filed with the application follows.

SEQUENCE LISTING (23 sequences)

SEQ ID NO: 1 - DNA, 29299 bp, Homo sapiens
cactcttgggtagaacgactctaacagcgaccgtctaaatgaaggtcacactaacaacgttcttaaacagattgtcttacttactagttggaactcgtcttctctaatactttttgaattatcgtaacatcgttacaccgacaattactttatgtcaaccgacgagggcgacaaaccgtggttggttggactgtgacagttgtagtgttatgctataaataagggttaataaaatgccgttgttgactttatgttacacaataattagtataaataatattcatagttaaactctttaaagactgtacggtcttctatttatccaaataatacttttcgtcaagacgaaccacgtacgaccgacgacgacacattatttatcggagacacccctttcaaaaaattttctttatttcgtttttttatcgtgacttttgtctttccttcgtagttttgagaagtttatggacgacacaggtaaccagttcgtgtaagtcctgtagcgtacggaaatcttgaggtcgtccaaggttgtcgatcatcctgtaagatctgaggaaaatcgggacagacaccgaagtcttattaaaggttgcgttggtaggtttaaaactgggtgtcgcacaatgtaaaccgtaacgccactgagtcaaggagtagaaatcacatgaggaagtattaaatctaattgaacacacttcgtgacttaggttatataccacagaaatccaggttggagtccagagggatgtacaacagtctttttctgtaaactcgtaaaattctcactttagttttcacgtgatggttccaaagattgtcgggtcaagacaggaccgaaaagaaggacgttgacaaaagtcgaacccactcagtgaaaagagagacctggaggtaaaagagtggggtgtagtgtcaggtcactcccgaagagaggtaggattttgaaagggggaccttgagttcagagagatacaacgggacgttttaatcgaagtcagggtatatgaaccgggctaatgggtgtctttcatgtcgttcgtagtagtaggtgtatcccagaggttttaaccgaaaggaccttggtaagtgttccggtaaagtcagtttcgggacccttttattggtcaaggaggttgacacagagtaacattttcttttgtctaataataacttgaatacattcgttggtataacggtatttaattcttataagtgtttatcaaatgtttaagatgtctttagtccgtctctctctttacacgaagtttaagataactgttctcatgtgagatgagttaacgatttccaacatttgtcgagttttctttttcacaagaggtctgagactttttgttttgtttttcttagtcgttacaaagtttcttggttttttttttttttttttttttagatttatacatatgtgtgtgtctgtgtttctaggttatcgtaaatggagttttgaaatcgatactttatcgttatctttgagtggtcaaatgtttgtccaagtgtaccgatttgataaaaacggggttatgtattagtttacttccgacacttggttttaaaccccatctcgtcaagagtaccgtcaaacgaaaaatttccggtatggaagggtctacggtttctcgtgatccaggtctatcgtggtgtctttttgtagtagatattggatgattagtccgggttgggacgaatcttgtcgtcgcatcctcagactgatgtaccttaaagtagaacggaagagtaagttgtcgtttgaggtctagggtttcttatgaccccggtccggttcacgtcaccgattgtggacgttagagtcgtgaaactctccgactacaccctcctggtgaactcaggttctcaatctctggtcggacccgttgtactacccttgaatagagaggtttttaatttttttttttttcgatccgtactaccgtacatggaaatgaggatcgatgaaccctccgactcgaccctcctagggaactcgggtcgtcaaggtccgatgtcactcggtactactgtgataacgtgaggtcggacccgttgtcgcattctaggacaggagaccggttttttcccagaccgtggacgaatcctcccgaaggttttgaaaaagtcgtttctatcactcaccgttttggatcgtacttcgggtctcatacaccgagacgcaatcataaagagtgtcgggtgacattactgacagtccaacgaaaattctaatactttcaggatataacttaacagtaagcttaactctggaacttcagacttctgccttaatgaacccttcttcgtagtgtcatagaatcttctcacagggaggtacttcgtctaaaccccagagtaaggcaaagacatgaatgtcattacctggtacaatccgttcagtaaattgtgtaaacctggggtcgaaggtttagatatgttaccttccatattaacctctctcatatttcggaaatcacgggtgaaatgaactctctaaaagtctcgtcagttactctgaaatctttattttcacttgaattttgtatttcacgaaatatttggggtcgtaacggacttcgggactctaacgaactaccgggtaacgcatataagtgtccgtgacggggttgaccgggaatgatgttgagatctttactgtccgtaagtaagaaggttaggtgtctactccgttgatgcttcacaataaaaattggggagtaaaaaattcctctttttgactcgaactcgtgtaattttttacaccgggtctcagttataccatatacaactggaaccttaagctcttttcagaagacagtgttctcgtcttcggtgtttgagtttatgaaaatcccaatacaatggttaacaccttgtgtacacgtactttactcgactcattctacggtttactggaccataacctctccgttatccctcaccaccccggacatcgtttgatctctctcgtaccgagtcaattttctctcaccgtcgttgagttgaggtcggttaacaacggtatgttataattcgggtccctaaagtcttgaagatcgatctttttatctccgatctatacatataaggacaagttttaacggagttaatcttctataatcgttcattaagtttacgttatgtgaaaacataatagtgatatgaccaggtggattattcccctgtcaaacgaaggacgagagtgtttcacaaagtctgattcaatactggtgaattcatacgtttctgttttgtcacatagtcattacgtcactaacactcgtacatgaagtctttgtttactagacccaagtttaggaccacaactgtaattcatcaaattattggagcccgttcagtgaactgaagagatatggagtcaaagggatagacattttaccttcattattctcatgaatgaggaaagtcaccaacactgatagtttacttaactgtatccattttgttaatcttgtcaaggactgtgtgccattctcagtacatttatagttacgaatactttcgagagtagggtcctattcgtagaggatcttttgtagaagcaggtacatggtctaattagtataaataagacgtcaactataaatacggtgtacaagaaagacccatctcttcggacttcaataagacaaataggactggaaccttttctgtttcgtcgagtacaggggtccctagatttttaaagtgacccttactagtgggtcacagaggttttggagtcggtcgtaaagagataagtgtcgacgtgacttctcgaaggaaggaccgaacacagaggttttcccctatgctaccgttccagacaaataatgagagtccgactacaccggcccctctacaccttaacacatcttaccttacgctaccttatactttaccacaccttatgtacacttgaagtacggacgaagagtccaaagaaggtgaaggggaaatacaccctgttctatcgacttcacccgacctcaacccaaaagaggaggaggtaaaccttccgacctcgaacgacctcaactcataaagaaaaggagtccagtcaatccaagactattttgggatcacccaatccgagaccaatctgtcgaaggggactcccgtctggggtgagactcgtcgttacggatctttactaccaagaagtttaggttcactattgggtatcattgattgagtaatcgaatcaagacggcatttcagtcttgtttcgttcctctttgtcttggagacgtcacttacctccttaaagactcccagtgaactttcgtctttgagttctcggggtaaaggttaaaggatgataacatgaactttatacctaaagtgtataaaccccattagtgaagtagtcatttcaaccggaagcattcaatttttgtgagtttaaaatctttgagttacaagacacccaatgtttactgacgggtggtacgacaccccgtactgtgggaaaacattaaagactttatgcttcatgataaaaaagaaattacgtaagagagaaaaatcaaagaggtaggacactatacagacaggttttcctgaagggtttttggtgacataccgtcttttccaaaagttttacgtactctcttaatatcgtttctctttattgagtgtgatttcaaaaattttatagaggcctgataccgatccttgataatgataccgattgttcacattaaagtcgtaaaaccctccggttccgtccgtctagggaattcagatcctcaaactctggtcgaacccgttacaccactttggggggagacgttttttatgttttattaatcgccccacaccaccacgtgtggacaccagggtcgatgagtacctccgattcctccctcctagtgaactcgggccctccgtctccaacgtcactcgattctaatacggtgacgtggggtcggaccctctgtctaagacagagttttttttttttttttagagacctgatatttgagagtacttagatcgtaataaacctagtctttatataagtatcctatctgacactactgtttatttagtttaaaccctacggagttgtgttctttataaaaatacatagtaatacattgtcaggtccctccgacttttatctcacatacaacgtccattctttaaaacgagacgtcagtaagtccttaacttcgactatcactaagacggtagaacttgtacaccgtagcgacagacagacctcccacggtagtgtcagtcgaaacctgtcgtggaacttacgatagtcccttcgatctcacaagaggacaagaaacgacaggaacggtcacagaagaggacttgagtgtagtcttcgtacggtcattcgtccaccatggtcgtcccaagattgggtccgtgaggttaagattccagttgaaacaatcacaatagattttttcttttcgttattatttaataggtgttcttttaaaatgttgagttcaaaaagtatgagaaatttttccgtaaaaaagtgtacatgagagtacaagatactaatctggattagtaacagtgaagtgccgatctctttgattctggtcttctcgaaggtctagaactgatcgtggtgagttactcaccctactggtcttgggacatgactagtacgtttgaagtggtgtattgtcgaacactataactcactcaacaaagtggatatgctggggagatttggttaaataattagatcttttacccttattatcgttaaagatacattattcaacaacctcgtgttctatttcaatatacatattttgtaaatcgtgtcaaggaccacgtattgtccagacatcatttataaacaacattaatcgtcgttttagtagagggagtaatgacgtcaactaaaaggaaataataacctttctttaaagagttgactcaaagtcaacttatgtcataatctaataaggaattgactcaaagtcgtaaaatttacatatgagggatgagttttgatggatgatttagtgcggacattaaggtcgtgagaccgtccggttccgcccacctagtactccagtcctctagttctggtaggaccgattgtgctactttggggtagagatgattttttacgtttttttaatcggtccgcaccaccgaccgtggacatcagggtcgatgaaccctccgactccgtcctcttaccacacttgggccctccgtctcgaacgtcacccggctctagcacggtgacgtggtgtcggacccgctgtctcactctgaggcagagtttttgtttgtttttttgtgtttttagatggatgatttttcttcaagaagttacgaatctgaaactcgtttctttttcagacgagattgtccttcgaccactatatctttccatttcaaagtgaagtgtccgtgaaactaaagggaagctccacctatgacttactaaacacacacgcgtgtaaaaagatacgtaataagttttaattttaaggaatctcctttggtgactttcggttagtaaatgttttgaaatttttactgtagaacttctcaagaaaccacgagtaagtagtttgaatcgttactaaattgacattaagaaataagtctaagtagagggtgttttatttttacggtatttcgaaatgtcatgacataggattacttatctctttgatttctttttcattctactcgttcactctccttttgggcttttactcggacaggaccgtacaaagatttttctttctttgtttgtttgttcgtcggggaggagagtcgagaaccctttctttataacttagaactgttatagacgtgaagtatcaactaagtatcgtactggatagagtttgttaaattctaagtttacttcaaacgttaattagaaagctatagtgaaacgttttgtaagagtattggaataggtcgggaaaatgtttagttaggacactccacttgtagtgacacaagggtaaaatgtctctttccgtgactcggtgtctctccaatatatgagtactagttattcgaccattctgattcttggtccttactatgacagaaggaagaggtttataggacaagaaataatactcatggatttgtcataatttttaattaatgtcgagttgttatcattcatttacaggagtacactttaggtggcaaattttgaattccaatagataaatagtttatttaatttaggatgagtgaattgttataagtaactcgagtaagacatttgttggtaatccggtccccgtctatactttatactccgagttagacactagtgtctctactttatatgttaaatctctctctttctattcgtactactgtttatttattacatacttttaatcggtaatagaatccggttgaaaaagattcgacattcgacagacggatgaagacggtccacaatcattaacaaaatttttcacccccttcttctcatgaagtaccacccttctataagtaactcctgtattcgtagaaggagaatctttaattgttacgtgtcaccggataacgttcaaaactttcgggacgtttgttattttcggactaatcaaaaataacttagtcatagaggatttgtgaaaaagtactttgttccaatgagtgtttagaacagctccttgattacaggatcctttcaccaaaagttcgaactcgtacatgtattcatagtaacctttccaacgtttttatgtttacacacccgaggtgaggtctttaagactaacttcaccagagtagacagtagactcttgaacgtaaaaacagtctaaggatcgactagactacaaagtcctgactcttgaattaaactcatcatagagatgtcttgtcaaaaattttacaagaggacctcatcctactaatatgaattgtttttacattatgtgagtccactacctgtgggaatcataggactaacctagtgatgtgtaatatatgtacattgtgtaaaagagttcatggggtatttaaacgtgtttatttatttatttattttaatatgaaaagagtttatttttttattttatttacaaggagaacttaccatcttagaaacaaaaaaacactattagtatttatgtatatttataagagtagtaatgtacgtacatcaatggaaggaaatgtactacgtggtctttcttatgggtgagattcttcctttcttacttctcttcttccgtaacaaattttctggataataatcttattcagtttaagatacagatggtaataattcgacaaactgaaactcgtccctaaccttccgtaaaatttaactccacctctatacgtgtttcggtgcaccctttacagtacacagggacgtatttctcttgttcgataaaacgaaccaacctctactcctctgtctccgacatgtattcttacacaagttaaatttcgttgttttatatagctggtttgatgaaactcgttagttcccctatataaccgagtgtagtgactttatatatgaccgtgtcgtctaaaggtcaatccagactagacgatcgagacaggggaggtcttatgtccgaggtccgtccgtccttccttctcctgtagtcaagagaaccacagatcgtgcgacggacataattccatccaggagttatttaagtacaacatcctttacttacgtacaagagtttctacgccaatgaaagtcatagtgacgaaaggagtaccaaaggtgaagttataatcagattgaacggaatccctgggttctaccgacgataagtgaagttaatcgatttgtgaagagaaaagtaccgacactctctgatcgatggagaaggtatttacttaaaagagaagaaagacccgtgttatcagagataaagggtcggagaaaatgttaatccacataggtacgttgagtcaagatcggttaccgcacactcatcatcactataggtggtgaacgtctggatgtgtatttccgagggtctgtgtagaagacacgagaaatgaccttgtgaacgaactaaggttatttatgtcgttggaatcgtcgatgtataacgtcaaccgtctcgaaagtacaaagtcgaagaagtataaaaaatcaaaacaacagtgacaaccaaaaaaaaaattaactaagtcctctactggattattttttaacttctttttatttcgtaaaacaagacctaaagagtaatccttgtactccaaatgagataacgttgaccgaatcaagtatactagtaggggactccactccctttttctacgcacttaactaattcggttccagtgtaccagctttacatcttaacccaaaactccagtcaaagggatttagtgggtctataggttcacctttagtccgaggtaactgttttcccttgtcaagaatctttacgttgatgtttacaggttagggtcaaccgttcaagcttcgttccttcccgaaaggtaatttcttacacctacgatggaccacccgttgacctccggtgaccgtatataaaaaaaaccccccccaaagtatttgataaccaaaaaaattaataataatatgaaattcaaaatcccatgtacacgtgttacacgtccaatcaatgtatacatatgcacacggtacgaccacacgacgtgggtaattgagtagtaaatcgtaatccatatagaggattacgatagggaggggggaggggggtggggtgttgtcaggggtctcacactacaaggggaaggacacaggtacacaaaagtaacaagtcaagggtggatactcactcttgtacgccacaaaccaaaaacaggaacgctatcaaatgactcttactactaaaggttaaagtaggtacagggatgtttcctgtacttgagtagtaaaaaataccgacgtatcataaggtaccacatatacacggtgtaagagaattaggtcagatagtaacaacctgtaaaccgaaccaaggttcagaaacgataacacttatcacggtgttatttgtatgcatacgtacacagaaatatcgtcgtactaaatatcaggaaacccatatatgggtcattaccctaccgacccagtttaccataaagatcaagatctagggactccttagcggtgtgactgaaggtgttaccaacttgatcaaatgtcagggtgattgtcacattttcacaaggataaagaggtgtaggagagctcgtggacaacaaaggactgaaaaattactaacggtaagattgaccacactctaccatagagtaacaccaaaactaaacgtaaagagactaccggtcactactactcgtaaaaaagtacacaaaaaaccgacgtatttacagaagaaaactcttcacagacaagtacaggaaacgggtgaaaaactaccccaacaaacaaaaaaagaacatttaaacaaactcaagtaacatctaagacctataatcgggaaacagtctactcatccaacacttttaaaagagggtaaaacatccaacggacaagtgagactaccatcaaagaaaacgacacgtcttcgagaagtcaaattaatctaggggaaacagttaaaacagaaaacaacggtaacgaaaaccacaaaatctgtacttcaggaacgggtacggatacaggacttaccattacggatccaaaagaagatcccaaaaataccaaaatccagattgtaaattcagaaattaggtagaacttaattaaaaacatattccacattccttccctaggtcaaagtcgaaagaggtataccgatcggtcaaaagggtcgtggtaaataatttatcccttaggaaaggggtaacgaacaaaaagagtccaaacagtttctagtctctcaacatctatacaccgcaataaagactcccgagacaagacaaggtaactagatatagagacaaaaccatggtcatggtacgacaaacccaatgacatcggaacatcatatcaaacttcagtccatcacactacggaggtcgaaacaagaaaaccgaatcctaactgaaccactacgcccgagaaaaaaccacggtatacttgaaatttcgtcaaaaaaggttaagacacttctttcagtaaccatcgaactacccctaccgtaacttagatatttaatggaacccgtcataccggtaaaagtgctataactaagaaggatgggtactcgtaccttacaagaaggtaaacaaacataggagaaaataaagtaactcgtcaccaaacatcaagaggaacttctcaaggaagtacagggaacattcaacctaaggatccataaaataagagaaacttcgttaacacttaccctcaagtgagtactaaaccgagagacaaacagacaacaaccacatattcttacgaagactaaaaacatgtaactaaaaatataggactctgaaacgacttcaacgaatagtcgaattcctctaaaacccgactctgttaccccaaaagatctatatgtacagtagacgtttgtccctgttaaactaaaggagaaaaggattaacttatgggaaataaaggaagaggacggattaacgggaccggtcttgaaggttgtggtacaacttatcctcaccactctctcccgtagggacagaacacggtcaaaagtttcccttacgaaggtcaaaaacgggtaagtcatactataaccgacacccaaaaagtatctattgagaataataaaactctatgcagggtagttatgaattaaataactctcaaaaaccgtacttctcaacaacttaaaacagtttccggaaaagacgtagataactctattagtacaccaaaaacagaaaccaagacaaatatacgacctaatgtaaataactaaacgaatataacttggtcggaacgtagggtccctacttcgggtgaactagtaccacctattcgaaaaactacacgacgacctaaaccaaactggtgaccgtataaaattcgtaccctcattgtgacagtccaaaaaatttaatgttttacgaaatcgtatctcttttaatatttcttgttatattcattgtctatacgtgagtgataggacgaattagtttacagtgtgaaacggttcgaactaagtttaaaaaatttcgtttctttgtaatgtctataccgacgttgtaggatacacggggtggcgactatgtatggagagaagggttcccattggtgaaagactgaaactatgaatagtaagggtccgtactaatttacgataacgacttaaacgtatatatgtatttattatatatgtcaacaaacgtacaagattttgaaacgtaatttattatagtttattaatttttaaaagtgtttaacgtaaaaattgagtcagaaaatattctaacggttattactatagagaagtctagtaagtaaaactgataatataataaaaagtaacatactgatacggtaccgagtgaataggtaagacaataactatttgtaaacacaacaaaggtgttaaaacgataattttattaccgtaacacttgtaagaacacacatatagtgacacatgtgtacgatctcaaagagattacataataccacatataacgacccggtttccgatacattcagaagttgaagggatctacagtatggttgagtatgtatatactggtcacactcgtaagagtcacgagatgtaacaggtctaagatgtacttcgtgaccaccggataaccagtccaactgactataatcttccaataacggtttcagatacactctctctgactcccagactttatggatctacattccctatatttcactctctcctttcttcaattgtataaatcctcgttttaggtgtactgaaacactaactaatacctcttttattcctcttcttcccttgtccttctgagagttcagaggtctaacttgtgttctccttcgaatacacggcactctgactactgtttaaggaaaacttgtatcacggaaactcccgaaccatcattttttctttcgtgataggtagtccgtaaacctataaatccagaccttctgacttttctctagttttgtcttttatgtttaatatcttagtagctctacccattttagtcttctcaacctagttcttttcatggatcttagtcatctcttcactcaattcttttatagagaccctttgtaattataaatttccatatattttccttctcttctgacacctcttctgtctctgacttcttcctctgttttacacagtatgacatcatcggtctccttatctcgaagtttcttactcaccagttggtgtaatttgtgtcgatcttttggttcttccatttctttacttttaatttgtaattgtatgttacttcaataactcaggtacaattttaccaaagttaccttatcgtagttacctttattaacgttaatcattttcttaaaatctttttcttttttaattatgtcgattgaaagagtttaatttaaaaaacttttattttgtcactctaccttaagctcacgttctacaaacaacttttagttgtgtgtactttcctttctctcacttggatttttttaaccgaggtctcagataattacatttctgatacaatataacagagagatagaaatccctttgtatatgggttaagtagaacacagtggtcttagtctaagtagtttgggtaagacctggtgagactagtgatcaaagtgggagtgtcagtatcatttctttgatttcgttttctgatgttctcgtttcctgtctttccctttacaataaaagaggggagtggaaacgggagaaactaaaagaggtaacaacgattttccttgtgaatcttttgatactttctttgaagacggacatttacgtcgaggtactaatacttaagacttaggaacattgtcttcttggttatcctgactaggtactgaagataatcatctctgacccttccatccactgaaatcgagtggttcggactagtgtcgttttatcttttactagtgtcacaggggaaaaataggaccccattgttacttgtaagtcaccctcggttgatgacataatttcaggacccacgtcgaggaccgtgtactgtaccgggtgttccatcatcaagactcatgggaacggatagtcaccacgaccccgctcttccctcccgtcggacgagtgatccctctcgtccttactccgatccttcatgtccctggaccgtttctacagaggacaaactctctctgaagtcaattacaagtcagttgaaggacaccacgattcttcactttcaacttgaactgatagttccttgtctccgtccaacaatcgacccggggaccctccttcagttgttcgaggtggtgtagactgttgtggatgacgaacgtcgggaagggggtccagtccgtcgacgtgtggagtacgaaggttgactcccccttacttacccatggttctcatccactcagatgaagaaagggtccccactcatcgcccacttctttagtcgtacatcacctgtaaatgtacacggcctatggagtatatacgtcacaccatagtaataggagtgacacgtctacttctgtgactccgagtccctgaacaagttctgtgtgtagaccagttatccctcggtcctaagttttagtgcagtcagatcatgagttcaggagacaagaaaggtgctgatgtaatctacatagggatctatcagatccacattgtcgtactcagagggtactttccttcacccccgagaaccttgtatggagaaatccttcggaaggtagtaacacgacggaaggaggagacacgtcggagtcgtgagtgacaactcgggaagagatcctcaaacgttagatgcccctcactacccgtgtattcctttattaaagttacatcataccgtttacgactcgatctatttacgcgcttactgatacttcttgtctcctaaccccagtggattgagttgtactctgagtaccttcagaggactcctctttggagactcaggatctctcactcttaaccggtctttttaattcttccccgtcccttaaggtctctcttcattgtccatttgttttcgtttctccgtattctatcagacctcagaccagtttaatgttagtcaaccttcatcatctcttattttatgtttcacctctctcccctcttcatttcgacttatctatttgtcccagtcgaatgtctcccaggatacgtccgatttaaggtctacgacgatatttttatgtcctttcttttgagtactttataaaattctaaaaacaccttataaaattctcgaaaacacttgtagagtacttcgtgaggacacaaacctccgtcgtgaccgtcgtttagtttgtattattttccagacatgtagtttgtaactgtgtaaataagttgttcgtgtataactcgtggatgatacaccgtccttgagagaagtagtcgttcataaaaccgtgatttattttgtgtcttgtgtggcgggagaaactttactgttatttcttttattcacttaatatataatagagtcgtctataacgtaccatatacctttcgtatagtcccttcccccacatttcacagtactctccttaatgttataattatcctacaattctgtcgaggatgacttcggtacaaatttgtctgtgaacctcctctcctccctcaaccgattcaactataaaccccattccgtaaggtccttccccctagtcggtcaagtttcgggaccccccacccccgacacgaaccgtataaactcctcaccattcctccggtcacaccgaccttgtcttactagtttctttttccaccatcatttactccagtctatttgtcattctctgttccctaaaaatccagtagatcttaaatctaaaaaaggactctcccgtctcctcggtgctctttcgagactctactcctactctactagattaagtccaaaattgacctatcaagtctcgttctcacccccgtcccttggtcactcctctgacaccgttattagtgcttttcaccacgtcgccgaacctggtccctcaatcgtcaccttcgtctctcttcactgttgtgagacgtataccctttcccacccgtcctctcttgtcacgggttctactaggtcataaaaccggactcttcgacccctttttctttgttgttgttgttgtagtcaccttccccaaagtccctcaggtccacaagaccaacgtcgaaacaaaacggaatttttataaactcatgcattgatcattaccctaacgacccaacttaccattaaggcaaaaatcaggaaactctttaacggtgtcacgaaaggaatcgtttgattccgtccttgtcttttggtttacggtgtacaagagtgaacattcaccctcgatttactattcttgagtacttgtgtatctccccttgttctctatgactccggatggactcccacctccaaccctcctccctctcctagtcctttttattgattactcgtgatccgaattatggacccactactttcatagacatattgtttcaggacactgcactcaaagggatccattgtttgaacgtgtacacggggacttgaattttattttgatatatgtatatatatgtataatctttcttaatatgaaaactcaaaattatcgtgtaaaagacattctaaaacgttaaatttgaagtgatataaaatatatttgttaattctcaactcaactggaactataatgtataatgtctataaaataattgtagataattaaaaattaataaactaaaaaagttttaaagtttattatatggataaaaagtctaaagtccgtccggtaacttttcgaggatcaagattaatgacaaggacattacgaaatacttatattgtcaggccggaaaggagaatctcaaacgtcagattccatctctttatattattttcttttacgtacttaaaaattgattataccacacccaagatttcgagtctatttaataaagcaaatcaagagtgttgttgggagactacgtccgtgataataaagggggtaaaattattactcctttgacttcgtgtctctcgaaccaactgaacgggttataatggtgtgagacacaccgattcgaccctaaacttggttcttttgagagaagggtatccagcaactttttaatactttccaattcggtggagagacgaacacaacggataaaggtggtacactcaggttacacaccactgtctcttcccatctacaaaccgtagacacttaagacacctaacacacagtactaagaaataaagacaggagacataggacttaacggtgatgggactcgtccactattctcattttaaggtaatgtaaccagaactcccctacccgtttgtgaaacctgagagaactataagatcaataatttataacgagtcgcattcaatctgttacttactctgaacaactacaaaagtaaagttaaacagaatattactagacacgagttgtacattttggttatctacattgtggaaaccttataaagactcatttgtaccccgtggttgagtttctcgttctccatttttacggatcacacctagttttagatgagatactgtcccttagagtacccgagacttcctaagaccagtgtatccctcatttatcgtctgagagttaagtctcagtctacactcaagtgtgcgttacaaaaccctgaagtaggacagaaaagggacgagaccctcagtattcttaattcaagattaggattaagacaacaatagatggactcactgtgattaatctatatattgaagagactccgagctgtaaatgtagatgtttatttcttccgatcttatgatttcggagaagataaagaaggttaataactaacatagccgagaatgagatatttaccaaagaagataaaatccctttaattaataaaacaagaataccacaacgacctggacaacgaaaagtaacgacattaatgaagagaaacaacttctggaaacggtctgctttacactacccacatattccgagaccgtaaaacgggtccagacatcgtgtatcttaaggtgattacccagacgacccgtagactctggtgtctcggtaaacagtattgtactgttaaggtcaacccgtccctatttacaatcgaaattgctaaaacctggtctcaaacagatctctctctcgtctcatgtttcggttttcgtagtagaaatctcgattcgtccgtactcaagtttagggttgggtcggtgaatgatctatacatcggtgtcggtggcggttcagagttaaatttacagtgaaagagtttgtccggaggatcccagagggtgcaaccgaatcaggtcttatgaccaaataggaatgccatattttaaataaggtagtaatacgtggtcataaattatttacgactccttacaccttgtttataaacaatttatttttcactgaattaggaagagacagagtcaggagtgaagtcacttcacccgttttcccatcttgttcaaaggacacgtttttcttagtccagtttcacgggatctttatcgtttgtgacagtgttgggatctatcgtactaatgttagactttatttgatcaagtttttcgtttagagtctgagttcaccccgaaaaagatcaaatcttgaacctcaatcttcttctttcttcccccgatttcacacgacgcacagatctacacggtccgtgacatgcattatcttacagtgtgtaaattataaacagattttcacactttcacacttaaaggtattctccctgtgtccaagaaccattttggttccaaacgagattgaaaagtgtgtgaaaccgtctgccaaaacggaaaaagaggattcaaccttgaaaactccggtaatgacggtcctcccttttcaatcactacgaatagatacaagtcttgatcttttaccggggaagaccaggggtcaaaccggggtaacaataagtgtacgacggatatttttctgttttggaggtcttccaccttttctacttatacgtcttacgatgtgtatctatgagtacatccactctaccgcttgtgtcgtctaaatccagatggttattctatgatggggtaaaccctactgtgtggaaggaatcttcactgtcaccgtcttgtatctgtttccctgattaattttcatacacccaagacgtctaacgtagacctcattctcaggtcactagatttaacatccggttccggagaacgaacgattgtaggagacagacggagtcaaaagaatggacgttttacctagtgacttgtagtgtaaagagaaataattaaataagtaagtgacttcttcgttcgacagtttttcgttgacgatgtatacagttctttctacggtctacgattttattttatgtttttaaactaatgatgtttaacgatggtagctcctcagtatcagattactttctctttttgtactctcacttattacttcagtcgtttttcaagttttctttttatttattttccgtatctataatttttacttcttcattttgatagaataagtctttcctatactaatacatgcctcttttagggtttcttagatgttgtagtctgagtagtcacttagatcgttctagtgacctatgtcaaatatatatttacaatagttattaacataaagacacggactgttgttttttaacttctgttgaaaattttgttgttacaaatattactgtggctttttatagtttaatcttcaagtacatttaacatcaaaggttctcgagggcgacctttaaccttcggtaacaactttatttaatttcttctaaattcgtttacctctctgaatggtaccaataccaagctttctgagatgtaacgattctacgttaaatgaggttttaacagatgtctaagttatgttaaagtcaatttcaaagactttgaaagtaaacaacaacaacaaaaaccttatctgttcgactaagacttcaaatatatgtttacgtttcctgcattttgtcgatttcttttaaacgtcttctttctttgattttcttaatgtgacagtctaaagctctggatgatgtttcgatgctaataattgtgtcacgtataaccatgttcttatccgtttatctgatttctttgtcttctgtctcaggtctttgacttgatgtgtatgtgctagtagactaaataatgtttccacggttccgttaactcatccttctcttgctacaagatgcatttaccgttataactcatagacataccattttttatttagaaccgatatacagtatattatacctgtttaattaatgtttacatcatatgtggtttacactttccattttgttttattgtacaatttttttcatatcatagaatggaaccctatcgtctataaagaatttgtcctgtgttcttcacttttccgttcggtgtcggagtgaaaacagaaggagtacggaagagaagatcacaccgagtcacgaatcacgtcctctttggtcattgggacttaacgtcgagaaggaagagtgatgtacttaagttaaaggagtagacagtttactcatatggttaagtatagagctttcgacaacgacactcttagtctattcgtattggagtgtcgaatacagataatcttgtcgtgaaccgtgtaccatttgtgaggtttcataaacaatttacttacttatctaattttccaccgtacaaaacatgatttgacaagttactatcacattttggtaaaccagtattacgcctttcccttcattccgccttaaggaaattagacacaaaatgcgtccaaggtttcctcgcaccacctctcttcctacgtctatcagacccactctcgatctccgacctcagtcgtccttcctgactccggcaaccacgaacccctcactcccgaggaaagacgagacaggatccgattcaaggggtgggtaaggaagaactctagatggagtttgtgtttagggagttaactggtgtcccccgcggggaagatacttaaaccgcgactatcgacactagacgggtcgtgtcaccccttttgtgttttaaatgtctagtccgtacaggcccgagtctaaggatgaggtcgtggaccaccggttccctggggttgacaatttatccgtaccactacggacgaaaggttcggacaaccctttctctctcccctcgcccctccttaccctctctctctctctgactcgttcgtacggttctgaattatatgaatataaatataattttctttatttatagtctactaatgttaaaccaacttgattctatgtgtcatcttataccttgattataggttatagtgtttcataagatcgctcggaaggatgtctttcttaacacccaccgacccctcatccgtaatcgatgatacactcacgtctcttatgagtcggaagaaggtctaccactcgatttcaagtttctagttcagtgcatgtgtggaagaaagagtagggtccaggatcagacgaacttaagtttaccggtaggtgtggaacggactttatgaacgttattaattctatgccgaaagacggacgaaccccaaaccaggtgttaagggaattctccggagtaaagttaatcctgagtgtgtagggaagttgtcattaaaacacagtccgaaccaatcgttgagttccgagttcgtatttaccctgtcttaagaaaaggaaaactttgagtggttatatcactaacatcgttgatcgatgtaacaaaaacaaaaaaaaaagggggagttaagattcgtgatacgtttccgaaatttcgtcaccagggttcggaaaaaccgtggtccctggtcaaaacaccttctgttaaaacacttttctgttttacaccttctggcacctgaccctaccaaacccctactaagttcgtgtaatgtaaacaacacgtgacacaaagataataataatgtaacataatatattactttattaatatgttgagtggtattacatcttagtcaccttcgggactcgaacaaaggacgttgatctgtgagggtagatccccactaccctctgccactgtccagtaatccgtaatctaagagtattcctcgcgtgttggatctagggagcgtacacgtcaagtactgtcccaaacacgacgatactcttaaattacggtgacgactagactgtcctccacctcgagtccgtcattccactcgttacccctcgtcgacatttattgcgactagagtgagtgggtgacgagtggaggacgacacaccgggtcaaggattgtccggtgttttaccatggacagacacaggggtcccaacccctggtgacggaatttccggaagtagagtaagtcaaaagtagttttaagacacaccatccatgagagtaatctgggtaaaatacccattccttgactccattttaaccaatatattgaacggattttattcagttcagagactactctcccggtcctaagttcaagttcgtcagactgaggttttagagtttcgtgaagacaccatcctttctctttacttaccttaccgtatctcagtagatttactgacgtcatccttccctcgtaaagggcacacgtcacaataaaaaaggcccgaaactttctatttatcctcgtacgtcaattttttctctcctcttccgtaagatccgtctttccggtcacgaatgtgtcttagagtcttaacattgtcaaggataatgtgggaccgtctcactacggttccgacaataacagttcgtgggaggacggagggtcaccccaactcttccccacttccctgtgaccgtcttcacttcgacccttcaaacgtgaacgatcaaccctgaacgtatcggtagaagagttacggtttctcctggagtcagagacacacgcgaaacaaaaaacaacaacaacaacaacaactaaacaccgggtccgatctcacgccaccacactagagacgagtgacgttggaggtagagggtccaagttccctaagaggacggaggtctgagggttcatcgaacctaatgtccgcgggcggtggtgtggacctattaaaaatatgaaaatcatccccacctcaaagtggcacaaccggtccgaccagacacacacgaaacctaaactctgtgagactactaaatctcaacttttaccctcatctaacccactaagagatcaatagtacaaatcagtttagtctaggcacgtaagttttagtattccgttcaaaaggacacaccgagtcattgtaggaatttctttatcaagactacaggtaggccacaaaaaagtctttctcgcagtcccaactgtcatcgacactacgaggtctacctcgacgcctattgtcgtatattcaaagtcccgtcaccaactccccgacaccctcccacccctcccttctacctactgaaaagagttggtagacataaactaaccttataacacactgaacactttatcttaatttctatactagaagaataccagaagagtgtcaaaagttccctaaaatcctcttttgcgaatcggtatgtctcgggttggaccattcaccgtcccgaccggtccagtcacgttgaagtttcagctacaacagtcacttacgaggtctacctaacgtctcttctggtttcaagtacagagccgtggaaagggttacatgtcccgaataacaaccctgtctcatcacggaccggatcttcaatttgtaagtaggtcgatcgataattccgaacttacggaagtttcttgtcgtacctaaaaagacacttagcactcgcaaaagcgttacgaattgtgccgtcgaccattactactaacgaggacaaagggaaacttaaagcacaagcaaatgaattgtcccgtaacgattagatcttcttccctcacccacttcttagggtaaacatttctcctatcgtccaattacttttcttcgtctccatacgcatccactatcacaaagatgttccgagccaagttaaccatactaaatttccgttcggaaccgaccgaccagtattattcccggtgtattacctcccctaaatgcaccgttaatggtaccaggaacgatcaccctatgttacaaaatcccgagggacctatgaattctaattacagacttagtcatcacaataacaacgttctagaatcacactaccctcggtacactccgtgcttaaaaatagggaatagtcttacattttatagagtatcagacgttcttgtggtcactgataccggacttcaacgggattctgtcaaatttgtaggacaactaacaaaacaaaaaaaaaggaaaaggaaccgttggtcttacgtacttactcagatcgcaatgaaaacaagtaggtccattatactaactttacccttaatatgtacaagttagtaaatctcttcttcctgatttttagtatctggatatcgtttaatttactaatatctcttagatggtacatttactgacgttaattcctgaagaagtacatggggcccggtctaagtgtcgtagaccctgtttgagaggtaccaaaaagggagccacataaataattcttactactaggacttgaagttcctctgaaccccttaaaaacctaaggacggtccatacatggaccggttctaattaaaccacttagtcttcaagggtccttggtatagtactcatgattctcttgtttaactaaatagatcatcatacaaagaggttgaatctatagacacgtttttttcacgtcgcctgtaccacgtgtaaggttcttcaagaggaggttccttcaccagttttatacattacgaataaataataggtaaaactctgggtttaataggtcagtcaccctagttatggaatgaggagaaggggtcttcggagtgtttatttcagaattgtggtagagttgtttttattctatccctggatctgtacctcttataccgacagagtacctaagattcgttagtccatctcataactctttacaataactttgtccttcaaggacgatttccacaaccaccctaaccctacggtcacgtctcactgtgtcataaacctgttcttgtgtattgtgctttcacagacttaggacaagaacagatattaccgtagaacggtaatttaggaaccgtgcacggacattagggtcgaagacccctccgacttcgtcctcttaacgaactttggccctccacctccaacgtcactcggccctagtgtggtgacgtgaggtcggacccactgtctcactctgagggagagttttttttttttttttttttttttttttttttctttttcctttttcttttttttcgttggtactctgctcgttcttcgattcaaatgtttatttacactaggtgtgaagagttgtagtcctgtccaggaagtacgaatctaaggtccagagaagaacgcttacccttgtcagtagtgaataggttactacgtaaattctcgtggttcaaaatttttctctgtttacagcttttctttacggtaaatagtagtttgtggtaataatttgtgatcgaacaaccgtatagacattcagaccaacagtaaaacgatccacctctcccgtcttaaaacctttcatagatccggtgtgggtacaaagtcttatcattcatgttttcggtgttacataactagtgaatctgagtagtatacaaacaggaaaataaaatttatggggttcctacctccagaaagatcggattaaaaggtcgattcttttagttcctattttttaaaagaacacaacaatgaaataggaatcatggggggacccttcatccatattaatcggagtagaatctctactcttttgactccgagtctctcctgacaggacattggtctttctcctacacaatcctagacttgggtagactgctttccgatacgagaattaatcattgtaaagggacggaacgttcctgtgtacatccagtgtcctatgggtcccttccatttacgagacaggaaaagagtggtcatgatgttgaatcattgtcggagaccgggttttactctgacctgtaactgaaattacctaccttcatgtgtaaggattgtacctaagtaagtcttcgtgggtctaaagtgttctcctttactactccgtaaaaagactccacaactttaacacgggaaacagtcagtgtttggttggtttttttttttttttccgaaacttttaaggagtttccattttccatcggaaagaagagagtatcaagactatatcagggttttcctttgttttcgaacgtattaagatcggggtcactaagaagaaaggaagaataattgatgtttagaagtggtgtaaaaaagaatgattaatcagtgtacgaattcgaggactcagtgcctcaacagatgaccaatatcgaacaagatcgagaaggtgggagtttaccttgaacgttccttaatccgggagacttctagcgtgtaagttcagtacttttgttcggttgttactttagttagtgacggctcttcccacctgttcgtgttcgtaattctgggtgatgacaactcagtcccggaagtctatacgacggttacccttcttctctctttttaatacaaataagtaaatatttatacacgtaagaacggaggtttccagggttaaagtgtgaccaggtcaacccaagagaaaggaaacgacgtaagtcctcgtgtcaacataaagtagatgacgaactcttacgtcacctcgaacagcggtcgtcactacctcggtttgtatttcggttaatggaaagggatccaccgattacctccgaggttcttcggtctcaaacgggtgtcggtataccaggctctcttatctggtacgtaaagacctccgaaatggactgaaagcggttttcgtacgtgtcttgcaccttgaaccggaggacttttccgcacagaagtcgaatccaataaggaaagagctacgagtggtactacagtccgaggatcatcctctcggtaattattggacggatagagtggtaatctgacacatgaagatcttccgtctttagaaaaagattactaaagaataaagggtcttgggaagccactgaaccgtaaactacccgttagaaccggtaggatttcgtaaggtacggtagtctatatgggacgtaacggtactcgaaatagtaaccgaaaatcttgtagtaggagggtgaaacttatttaccagatcgtctgttatgtcagggaacacggtccgttgtaagacctacgaaatacatgtaatcgagtaacttagtaaagttaagttagtaagttgcgtccccaaacttagaatcgacaaactccagtaacaggtacgtgagtggatattgtaacaagacagagaaagacgtttacattctatttttataatggaagtaagatcttttgtggggaaacatcttatccaaatatggaagtccgtacacctgaaaggttaggtttgaggtcctcatctgtctatgggtggtcctgatccgttacgtccttttagagtccgaagtcgatcctgacaaagtatgttaaaggacgtaccggtccttgttcccacttccgtacgtgagacactcgtcgggtaaacacctgtcacccagtaccctgacttccttggtacaatgtgtacggactcaaaagaaaggttcgagtctttggtatagcttgtggggagggaacccctcttcactcactcgtccacctctctgctatcattacaatcataccaccttgaagaaggggtatctacctttgtgactcccgattcttcttcccggagaggaggttgtacacaatagatcgttccgaccaagataaattcttactatatatcagatcacattatcttatgttatacggatcgagattttaatacaacctttttttagttgtaatgctacacgatataagtcagttactcatttataaagacacggacggtgtacgagtcgtaatattaatctcggtggcactttttatgaataggcactaggaaatacgacagtttcggatttaaggggtgaattggttcttaggacctattaagggttttttgtttaaataataaacaaagataccaacacacaaacagtttttaacttcgtaattatctttattcttgttaaatctgatattttcggtatccgaatatttttacgatcgtagtcgtgtaaggttttgacggacggggtagggaactaccatacacactaacgacagtgttttgatcgtcaatcttagaaaacattgactcctatatttggtttaaatctttatacagaaatgatttcccacctttgaatctttgacttcacctaaatggtgttacttgatcttgatttacatggttgtgtccgagttttgtgagattctattaaaaagtttaaataaattttaattcttttcttttgacccattgtaacttagtgtttgtcaacttttgtgaccccaatgtatcataattgtatattaatgtactagtaaacactatttgtcttttaaatttttttctttttcctctttttttattttttatttctttttgttttttgtttttttatcttttactttactctttttttaactagttaccgtttagtgacctctatttagtaacacatgtctaaagggataactttttttattgttattaatttgtggtcgattcggaagaaagaagaaaactaaaaacactttttagcgttattctacatagagatctagcacacgaacggtcttagaaacgacaaagaatccactttctagtaactattcttagaccgtacctcttgtcagttccttcgtaacgtcgagttatgttttgccaccggtcccttctaggtgacttaatcctcagtcgtcagtaataagatgatggacgattagaagatactcgaagcagttcagtaaattcgaaccatgggcagtcaaaggagtagacttttgactcttttcaacaaagtttaacagattcaggtaaggtcgaactagtatgatcgtagaatacacgtcgaagaatttcaggtcgagtgtggagacagttgagggacatattatactgaaggtttttttgtggacaccaaaccaatatgtatatatacctgtatatatacaatatgtatatataaccaatatggatat

SEQ ID NO: 2 - DNA, 25265 bp, Homo sapiens
cactcttgggtagaacgactctaacagcgaccgtctaaatgaaggtcacactaacaacgttcttaaacagattgtcttacttactagttggaactcgtcttctctaatactttttgaattatcgtaacatcgttacaccgacaattactttatgtcaaccgacgagggcgacaaaccgtggttggttggactgtgacagttgtagtgttatgctataaataagggttaataaaatgccgttgttgactttatgttacacaataattagtataaataatattcatagttaaactctttaaagactgtacggtcttctatttatccaaataatacttttcgtcaagacgaaccacgtacgaccgacgacgacacattatttatcggagacacccctttcaaaaaattttctttatttcgtttttttatcgtgacttttgtctttccttcgtagttttgagaagtttatggacgacacaggtaaccagttcgtgtaagtcctgtagcgtacggaaatcttgaggtcgtccaaggttgtcgatcatcctgtaagatctgaggaaaatcgggacagacaccgaagtcttattaaaggttgcgttggtaggtttaaaactgggtgtcgcacaatgtaaaccgtaacgccactgagtcaaggagtagaaatcacatgaggaagtattaaatctaattgaacacacttcgtgacttaggttatataccacagaaatccaggttggagtccagagggatgtacaacagtctttttctgtaaactcgtaaaattctcactttagttttcacgtgatggttccaaagattgtcgggtcaagacaggaccgaaaagaaggacgttgacaaaagtcgaacccactcagtgaaaagagagacctggaggtaaaagagtggggtgtagtgtcaggtcactcccgaagagaggtaggattttgaaagggggaccttgagttcagagagatacaacgggacgttttaatcgaagtcagggtatatgaaccgggctaatgggtgtctttcatgtcgttcgtagtagtaggtgtatcccagaggttttaaccgaaaggaccttggtaagtgttccggtaaagtcagtttcgggacccttttattggtcaaggaggttgacacagagtaacattttcttttgtctaataataacttgaatacattcgttggtataacggtatttaattcttataagtgtttatcaaatgtttaagatgtctttagtccgtctctctctttacacgaagtttaagataactgttctcatgtgagatgagttaacgatttccaacatttgtcgagttttctttttcacaagaggtctgagactttttgttttgtttttcttagtcgttacaaagtttcttggttttttttttttttttttttttagatttatacatatgtgtgtgtctgtgtttctaggttatcgtaaatggagttttgaaatcgatactttatcgttatctttgagtggtcaaatgtttgtccaagtgtaccgatttgataaaaacggggttatgtattagtttacttccgacacttggttttaaaccccatctcgtcaagagtaccgtcaaacgaaaaatttccggtatggaagggtctacggtttctcgtgatccaggtctatcgtggtgtctttttgtagtagatattggatgattagtccgggttgggacgaatcttgtcgtcgcatcctcagactgatgtaccttaaagtagaacggaagagtaagttgtcgtttgaggtctagggtttcttatgaccccggtccggttcacgtcaccgattgtggacgttagagtcgtgaaactctccgactacaccctcctggtgaactcaggttctcaatctctggtcggacccgttgtactacccttgaatagagaggtttttaatttttttttttttcgatccgtactaccgtacatggaaatgaggatcgatgaaccctccgactcgaccctcctagggaactcgggtcgtcaaggtccgatgtcactcggtactactgtgataacgtgaggtcggacccgttgtcgcattctaggacaggagaccggttttttcccagaccgtggacgaatcctcccgaaggttttgaaaaagtcgtttctatcactcaccgttttggatcgtacttcgggtctcatacaccgagacgcaatcataaagagtgtcgggtgacattactgacagtccaacgaaaattctaatactttcaggatataacttaacagtaagcttaactctggaacttcagacttctgccttaatgaacccttcttcgtagtgtcatagaatcttctcacagggaggtacttcgtctaaaccccagagtaaggcaaagacatgaatgtcattacctggtacaatccgttcagtaaattgtgtaaacctggggtcgaaggtttagatatgttaccttccatattaacctctctcatatttcggaaatcacgggtgaaatgaactctctaaaagtctcgtcagttactctgaaatctttattttcacttgaattttgtatttcacgaaatatttggggtcgtaacggacttcgggactctaacgaactaccgggtaacgcatataagtgtccgtgacggggttgaccgggaatgatgttgagatctttactgtccgtaagtaagaaggttaggtgtctactccgttgatgcttcacaataaaaattggggagtaaaaaattcctctttttgactcgaactcgtgtaattttttacaccgggtctcagttataccatatacaactggaaccttaagctcttttcagaagacagtgttctcgtcttcggtgtttgagtttatgaaaatcccaatacaatggttaacaccttgtgtacacgtactttactcgactcattctacggtttactggaccataacctctccgttatccctcaccaccccggacatcgtttgatctctctcgtaccgagtcaattttctctcaccgtcgttgagttgaggtcggttaacaacggtatgttataattcgggtccctaaagtcttgaagatcgatctttttatctccgatctatacatataaggacaagttttaacggagttaatcttctataatcgttcattaagtttacgttatgtgaaaacataatagtgatatgaccaggtggattattcccctgtcaaacgaaggacgagagtgtttcacaaagtctgattcaatactggtgaattcatacgtttctgttttgtcacatagtcattacgtcactaacactcgtacatgaagtctttgtttactagacccaagtttaggaccacaactgtaattcatcaaattattggagcccgttcagtgaactgaagagatatggagtcaaagggatagacattttaccttcattattctcatgaatgaggaaagtcaccaacactgatagtttacttaactgtatccattttgttaatcttgtcaaggactgtgtgccattctcagtacatttatagttacgaatactttcgagagtagggtcctattcgtagaggatcttttgtagaagcaggtacatggtctaattagtataaataagacgtcaactataaatacggtgtacaagaaagacccatctcttcggacttcaataagacaaataggactggaaccttttctgtttcgtcgagtacaggggtccctagatttttaaagtgacccttactagtgggtcacagaggttttggagtcggtcgtaaagagataagtgtcgacgtgacttctcgaaggaaggaccgaacacagaggttttcccctatgctaccgttccagacaaataatgagagtccgactacaccggcccctctacaccttaacacatcttaccttacgctaccttatactttaccacaccttatgtacacttgaagtacggacgaagagtccaaagaaggtgaaggggaaatacaccctgttctatcgacttcacccgacctcaacccaaaagaggaggaggtaaaccttccgacctcgaacgacctcaactcataaagaaaaggagtccagtcaatccaagactattttgggatcacccaatccgagaccaatctgtcgaaggggactcccgtctggggtgagactcgtcgttacggatctttactaccaagaagtttaggttcactattgggtatcattgattgagtaatcgaatcaagacggcatttcagtcttgtttcgttcctctttgtcttggagacgtcacttacctccttaaagactcccagtgaactttcgtctttgagttctcggggtaaaggttaaaggatgataacatgaactttatacctaaagtgtataaaccccattagtgaagtagtcatttcaaccggaagcattcaatttttgtgagtttaaaatctttgagttacaagacacccaatgtttactgacgggtggtacgacaccccgtactgtgggaaaacattaaagactttatgcttcatgataaaaaagaaattacgtaagagagaaaaatcaaagaggtaggacactatacagacaggttttcctgaagggtttttggtgacataccgtcttttccaaaagttttacgtactctcttaatatcgtttctctttattgagtgtgatttcaaaaattttatagaggcctgataccgatccttgataatgataccgattgttcacattaaagtcgtaaaaccctccggttccgtccgtctagggaattcagatcctcaaactctggtcgaacccgttacaccactttggggggagacgttttttatgttttattaatcgccccacaccaccacgtgtggacaccagggtcgatgagtacctccgattcctccctcctagtgaactcgggccctccgtctccaacgtcactcgattctaatacggtgacgtggggtcggaccctctgtctaagacagagttttttttttttttttagagacctgatatttgagagtacttagatcgtaataaacctagtctttatataagtatcctatctgacactactgtttatttagtttaaaccctacggagttgtgttctttataaaaatacatagtaatacattgtcaggtccctccgacttttatctcacatacaacgtccattctttaaaacgagacgtcagtaagtccttaacttcgactatcactaagacggtagaacttgtacaccgtagcgacagacagacctcccacggtagtgtcagtcgaaacctgtcgtggaacttacgatagtcccttcgatctcacaagaggacaagaaacgacaggaacggtcacagaagaggacttgagtgtagtcttcgtacggtcattcgtccaccatggtcgtcccaagattgggtccgtgaggttaagattccagttgaaacaatcacaatagattttttcttttcgttattatttaataggtgttcttttaaaatgttgagttcaaaaagtatgagaaatttttccgtaaaaaagtgtacatgagagtacaagatactaatctggattagtaacagtgaagtgccgatctctttgattctggtcttctcgaaggtctagaactgatcgtggtgagttactcaccctactggtcttgggacatgactagtacgtttgaagtggtgtattgtcgaacactataactcactcaacaaagtggatatgctggggagatttggttaaataattagatcttttacccttattatcgttaaagatacattattcaacaacctcgtgttctatttcaatatacatattttgtaaatcgtgtcaaggaccacgtattgtccagacatcatttataaacaacattaatcgtcgttttagtagagggagtaatgacgtcaactaaaaggaaataataacctttctttaaagagttgactcaaagtcaacttatgtcataatctaataaggaattgactcaaagtcgtaaaatttacatatgagggatgagttttgatggatgatttagtgcggacattaaggtcgtgagaccgtccggttccgcccacctagtactccagtcctctagttctggtaggaccgattgtgctactttggggtagagatgattttttacgtttttttaatcggtccgcaccaccgaccgtggacatcagggtcgatgaaccctccgactccgtcctcttaccacacttgggccctccgtctcgaacgtcacccggctctagcacggtgacgtggtgtcggacccgctgtctcactctgaggcagagtttttgtttgtttttttgtgtttttagatggatgatttttcttcaagaagttacgaatctgaaactcgtttctttttcagacgagattgtccttcgaccactatatctttccatttcaaagtgaagtgtccgtgaaactaaagggaagctccacctatgacttactaaacacacacgcgtgtaaaaagatacgtaataagttttaattttaaggaatctcctttggtgactttcggttagtaaatgttttgaaatttttactgtagaacttctcaagaaaccacgagtaagtagtttgaatcgttactaaattgacattaagaaataagtctaagtagagggtgttttatttttacggtatttcgaaatgtcatgacataggattacttatctctttgatttctttttcattctactcgttcactctccttttgggcttttactcggacaggaccgtacaaagatttttctttctttgtttgtttgttcgtcggggaggagagtcgagaaccctttctttataacttagaactgttatagacgtgaagtatcaactaagtatcgtactggatagagtttgttaaattctaagtttacttcaaacgttaattagaaagctatagtgaaacgttttgtaagagtattggaataggtcgggaaaatgtttagttaggacactccacttgtagtgacacaagggtaaaatgtctctttccgtgactcggtgtctctccaatatatgagtactagttattcgaccattctgattcttggtccttactatgacagaaggaagaggtttataggacaagaaataatactcatggatttgtcataatttttaattaatgtcgagttgttatcattcatttacaggagtacactttaggtggcaaattttgaattccaatagataaatagtttatttaatttaggatgagtgaattgttataagtaactcgagtaagacatttgttggtaatccggtccccgtctatactttatactccgagttagacactagtgtctctactttatatgttaaatctctctctttctattcgtactactgtttatttattacatacttttaatcggtaatagaatccggttgaaaaagattcgacattcgacagacggatgaagacggtccacaatcattaacaaaatttttcacccccttcttctcatgaagtaccacccttctataagtaactcctgtattcgtagaaggagaatctttaattgttacgtgtcaccggataacgttcaaaactttcgggacgtttgttattttcggactaatcaaaaataacttagtcatagaggatttgtgaaaaagtactttgttccaatgagtgtttagaacagctccttgattacaggatcctttcaccaaaagttcgaactcgtacatgtattcatagtaacctttccaacgtttttatgtttacacacccgaggtgaggtctttaagactaacttcaccagagtagacagtagactcttgaacgtaaaaacagtctaaggatcgactagactacaaagtcctgactcttgaattaaactcatcatagagatgtcttgtcaaaaattttacaagaggacctcatcctactaatatgaattgtttttacattatgtgagtccactacctgtgggaatcataggactaacctagtgatgtgtaatatatgtacattgtgtaaaagagttcatggggtatttaaacgtgtttatttatttatttattttaatatgaaaagagtttatttttttattttatttacaaggagaacttaccatcttagaaacaaaaaaacactattagtatttatgtatatttataagagtagtaatgtacgtacatcaatggaaggaaatgtactacgtggtctttcttatgggtgagattcttcctttcttacttctcttcttccgtaacaaattttctggataataatcttattcagtttaagatacagatggtaataattcgacaaactgaaactcgtccctaaccttccgtaaaatttaactccacctctatacgtgtttcggtgcaccctttacagtacacagggacgtatttctcttgttcgataaaacgaaccaacctctactcctctgtctccgacatgtattcttacacaagttaaatttcgttgttttatatagctggtttgatgaaactcgttagttcccctatataaccgagtgtagtgactttatatatgaccgtgtcgtctaaaggtcaatccagactagacgatcgagacaggggaggtcttatgtccgaggtccgtccgtccttccttctcctgtagtcaagagaaccacagatcgtgcgacggacataattccatccaggagttatttaagtacaacatcctttacttacgtacaagagtttctacgccaatgaaagtcatagtgacgaaaggagtaccaaaggtgaagttataatcagattgaacggaatccctgggttctaccgacgataagtgaagttaatcgatttgtgaagagaaaagtaccgacactctctgatcgatggagaaggtatttacttaaaagagaagaaagacccgtgttatcagagataaagggtcggagaaaatgttaatccacataggtacgttgagtcaagatcggttaccgcacactcatcatcactataggtggtgaacgtctggatgtgtatttccgagggtctgtgtagaagacacgagaaatgaccttgtgaacgaactaaggttatttatgtcgttggaatcgtcgatgtataacgtcaaccgtctcgaaagtacaaagtcgaagaagtataaaaaatcaaaacaacagtgacaaccaaaaaaaaaattaactaagtcctctactggattattttttaacttctttttatttcgtaaaacaagacctaaagagtaatccttgtactccaaatgagataacgttgaccgaatcaagtatactagtaggggactccactccctttttctacgcacttaactaattcggttccagtgtaccagctttacatcttaacccaaaactccagtcaaagggatttagtgggtctataggttcacctttagtccgaggtaactgttttcccttgtcaagaatctttacgttgatgtttacaggttagggtcaaccgttcaagcttcgttccttcccgaaaggtaatttcttacacctacgatggaccacccgttgacctccggtgaccgtatataaaaaaaaccccccccaaagtatttgataaccaaaaaaattaataataatatgaaattcaaaatcccatgtacacgtgttacacgtccaatcaatgtatacatatgcacacggtacgaccacacgacgtgggtaattgagtagtaaatcgtaatccatatagaggattacgatagggaggggggaggggggtggggtgttgtcaggggtctcacactacaaggggaaggacacaggtacacaaaagtaacaagtcaagggtggatactcactcttgtacgccacaaaccaaaaacaggaacgctatcaaatgactcttactactaaaggttaaagtaggtacagggatgtttcctgtacttgagtagtaaaaaataccgacgtatcataaggtaccacatatacacggtgtaagagaattaggtcagatagtaacaacctgtaaaccgaaccaaggttcagaaacgataacacttatcacggtgttatttgtatgcatacgtacacagaaatatcgtcgtactaaatatcaggaaacccatatatgggtcattaccctaccgacccagtttaccataaagatcaagatctagggactccttagcggtgtgactgaaggtgttaccaacttgatcaaatgtcagggtgattgtcacattttcacaaggataaagaggtgtaggagagctcgtggacaacaaaggactgaaaaattactaacggtaagattgaccacactctaccatagagtaacaccaaaactaaacgtaaagagactaccggtcactactactcgtaaaaaagtacacaaaaaaccgacgtatttacagaagaaaactcttcacagacaagtacaggaaacgggtgaaaaactaccccaacaaacaaaaaaagaacatttaaacaaactcaagtaacatctaagacctataatcgggaaacagtctactcatccaacacttttaaaagagggtaaaacatccaacggacaagtgagactaccatcaaagaaaacgacacgtcttcgagaagtcaaattaatctaggggaaacagttaaaacagaaaacaacggtaacgaaaaccacaaaatctgtacttcaggaacgggtacggatacaggacttaccattacggatccaaaagaagatcccaaaaataccaaaatccagattgtaaattcagaaattaggtagaacttaattaaaaacatattccacattccttccctaggtcaaagtcgaaagaggtataccgatcggtcaaaagggtcgtggtaaataatttatcccttaggaaaggggtaacgaacaaaaagagtccaaacagtttctagtctctcaacatctatacaccgcaataaagactcccgagacaagacaaggtaactagatatagagacaaaaccatggtcatggtacgacaaacccaatgacatcggaacatcatatcaaacttcagtccatcacactacggaggtcgaaacaagaaaaccgaatcctaactgaaccactacgcccgagaaaaaaccacggtatacttgaaatttcgtcaaaaaaggttaagacacttctttcagtaaccatcgaactacccctaccgtaacttagatatttaatggaacccgtcataccggtaaaagtgctataactaagaaggatgggtactcgtaccttacaagaaggtaaacaaacataggagaaaataaagtaactcgtcaccaaacatcaagaggaacttctcaaggaagtacagggaacattcaacctaaggatccataaaataagagaaacttcgttaacacttaccctcaagtgagtactaaaccgagagacaaacagacaacaaccacatattcttacgaagactaaaaacatgtaactaaaaatataggactctgaaacgacttcaacgaatagtcgaattcctctaaaacccgactctgttaccccaaaagatctatatgtacagtagacgtttgtccctgttaaactaaaggagaaaaggattaacttatgggaaataaaggaagaggacggattaacgggaccggtcttgaaggttgtggtacaacttatcctcaccactctctcccgtagggacagaacacggtcaaaagtttcccttacgaaggtcaaaaacgggtaagtcatactataaccgacacccaaaaagtatctattgagaataataaaactctatgcagggtagttatgaattaaataactctcaaaaaccgtacttctcaacaacttaaaacagtttccggaaaagacgtagataactctattagtacaccaaaaacagaaaccaagacaaatatacgacctaatgtaaataactaaacgaatataacttggtcggaacgtagggtccctacttcgggtgaactagtaccacctattcgaaaaactacacgacgacctaaaccaaactggtgaccgtataaaattcgtaccctcattgtgacagtccaaaaaatttaatgttttacgaaatcgtatctcttttaatatttcttgttatattcattgtctatacgtgagtgataggacgaattagtttacagtgtgaaacggttcgaactaagtttaaaaaatttcgtttctttgtaatgtctataccgacgttgtaggatacacggggtggcgactatgtatggagagaagggttcccattggtgaaagactgaaactatgaatagtaagggtccgtactaatttacgataacgacttaaacgtatatatgtatttattatatatgtcaacaaacgtacaagattttgaaacgtaatttattatagtttattaatttttaaaagtgtttaacgtaaaaattgagtcagaaaatattctaacggttattactatagagaagtctagtaagtaaaactgataatataataaaaagtaacatactgatacggtaccgagtgaataggtaagacaataactatttgtaaacacaacaaaggtgttaaaacgataattttattaccgtaacacttgtaagaacacacatatagtgacacatgtgtacgatctcaaagagattacataataccacatataacgacccggtttccgatacattcagaagttgaagggatctacagtatggttgagtatgtatatactggtcacactcgtaagagtcacgagatgtaacaggtctaagatgtacttcgtgaccaccggataaccagtccaactgactataatcttccaataacggtttcagatacactctctctgactcccagactttatggatctacattccctatatttcactctctcctttcttcaattgtataaatcctcgttttaggtgtactgaaacactaactaatacctcttttattcctcttcttcccttgtccttctgagagttcagaggtctaacttgtgttctccttcgaatacacggcactctgactactgtttaaggaaaacttgtatcacggaaactcccgaaccatcattttttctttcgtgataggtagtccgtaaacctataaatccagaccttctgacttttctctagttttgtcttttatgtttaatatcttagtagctctacccattttagtcttctcaacctagttcttttcatggatcttagtcatctcttcactcaattcttttatagagaccctttgtaattataaatttccatatattttccttctcttctgacacctcttctgtctctgacttcttcctctgttttacacagtatgacatcatcggtctccttatctcgaagtttcttactcaccagttggtgtaatttgtgtcgatcttttggttcttccatttctttacttttaatttgtaattgtatgttacttcaataactcaggtacaattttaccaaagttaccttatcgtagttacctttattaacgttaatcattttcttaaaatctttttcttttttaattatgtcgattgaaagagtttaatttaaaaaacttttattttgtcactctaccttaagctcacgttctacaaacaacttttagttgtgtgtactttcctttctctcacttggatttttttaaccgaggtctcagataattacatttctgatacaatataacagagagatagaaatccctttgtatatgggttaagtagaacacagtggtcttagtctaagtagtttgggtaagacctggtgagactagtgatcaaagtgggagtgtcagtatcatttctttgatttcgttttctgatgttctcgtttcctgtctttccctttacaataaaagaggggagtggaaacgggagaaactaaaagaggtaacaacgattttccttgtgaatcttttgatactttctttgaagacggacatttacgtcgaggtactaatacttaagacttaggaacattgtcttcttggttatcctgactaggtactgaagataatcatctctgacccttccatccactgaaatcgagtggttcggactagtgtcgttttatcttttactagtgtcacaggggaaaaataggaccccattgttacttgtaagtcaccctcggttgatgacataatttcaggacccacgtcgaggaccgtgtactgtaccgggtgttccatcatcaagactcatgggaacggatagtcaccacgaccccgctcttccctcccgtcggacgagtgatccctctcgtccttactccgatccttcatgtccctggaccgtttctacagaggacaaactctctctgaagtcaattacaagtcagttgaaggacaccacgattcttcactttcaacttgaactgatagttccttgtctccgtccaacaatcgacccggggaccctccttcagttgttcgaggtggtgtagactgttgtggatgacgaacgtcgggaagggggtccagtccgtcgacgtgtggagtacgaaggttgactcccccttacttacccatggttctcatccactcagatgaagaaagggtccccactcatcgcccacttctttagtcgtacatcacctgtaaatgtacacggcctatggagtatatacgtcacaccatagtaataggagtgacacgtctacttctgtgactccgagtccctgaacaagttctgtgtgtagaccagttatccctcggtcctaagttttagtgcagtcagatcatgagttcaggagacaagaaaggtgctgatgtaatctacatagggatctatcagatccacattgtcgtactcagagggtactttccttcacccccgagaaccttgtatggagaaatccttcggaaggtagtaacacgacggaaggaggagacacgtcggagtcgtgagtgacaactcgggaagagatcctcaaacgttagatgcccctcactacccgtgtattcctttattaaagttacatcataccgtttacgactcgatctatttacgcgcttactgatacttcttgtctcctaaccccagtggattgagttgtactctgagtaccttcagaggactcctctttggagactcaggatctctcactcttaaccggtctttttaattcttccccgtcccttaaggtctctcttcattgtccatttgttttcgtttctccgtattctatcagacctcagaccagtttaatgttagtcaaccttcatcatctcttattttatgtttcacctctctcccctcttcatttcgacttatctatttgtcccagtcgaatgtctcccaggatacgtccgatttaaggtctacgacgatatttttatgtcctttcttttgagtactttataaaattctaaaaacaccttataaaattctcgaaaacacttgtagagtacttcgtgaggacacaaacctccgtcgtgaccgtcgtttagtttgtattattttccagacatgtagtttgtaactgtgtaaataagttgttcgtgtataactcgtggatgatacaccgtccttgagagaagtagtcgttcataaaaccgtgatttattttgtgtcttgtgtggcgggagaaactttactgttatttcttttattcacttaatatataatagagtcgtctataacgtaccatatacctttcgtatagtcccttcccccacatttcacagtactctccttaatgttataattatcctacaattctgtcgaggatgacttcggtacaaatttgtctgtgaacctcctctcctccctcaaccgattcaactataaaccccattccgtaaggtccttccccctagtcggtcaagtttcgggaccccccacccccgacacgaaccgtataaactcctcaccattcctccggtcacaccgaccttgtcttactagtttctttttccaccatcatttactccagtctatttgtcattctctgttccctaaaaatccagtagatcttaaatctaaaaaaggactctcccgtctcctcggtgctctttcgagactctactcctactctactagattaagtccaaaattgacctatcaagtctcgttctcacccccgtcccttggtcactcctctgacaccgttattagtgcttttcaccacgtcgccgaacctggtccctcaatcgtcaccttcgtctctcttcactgttgtgagacgtataccctttcccacccgtcctctcttgtcacgggttctactaggtcataaaaccggactcttcgacccctttttctttgttgttgttgttgtagtcaccttccccaaagtccctcaggtccacaagaccaacgtcgaaacaaaacggaatttttataaactcatgcattgatcattaccctaacgacccaacttaccattaaggcaaaaatcaggaaactctttaacggtgtcacgaaaggaatcgtttgattccgtccttgtcttttggtttacggtgtacaagagtgaacattcaccctcgatttactattcttgagtacttgtgtatctccccttgttctctatgactccggatggactcccacctccaaccctcctccctctcctagtcctttttattgattactcgtgatccgaattatggacccactactttcatagacatattgtttcaggacactgcactcaaagggatccattgtttgaacgtgtacacggggacttgaattttattttgatatatgtatatatatgtataatctttcttaatatgaaaactcaaaattatcgtgtaaaagacattctaaaacgttaaatttgaagtgatataaaatatatttgttaattctcaactcaactggaactataatgtataatgtctataaaataattgtagataattaaaaattaataaactaaaaaagttttaaagtttattatatggataaaaagtctaaagtccgtccggtaacttttcgaggatcaagattaatgacaaggacattacgaaatacttatattgtcaggccggaaaggagaatctcaaacgtcagattccatctctttatattattttcttttacgtacttaaaaattgattataccacacccaagatttcgagtctatttaataaagcaaatcaagagtgttgttgggagactacgtccgtgataataaagggggtaaaattattactcctttgacttcgtgtctctcgaaccaactgaacgggttataatggtgtgagacacaccgattcgaccctaaacttggttcttttgagagaagggtatccagcaactttttaatactttccaattcggtggagagacgaacacaacggataaaggtggtacactcaggttacacaccactgtctcttcccatctacaaaccgtagacacttaagacacctaacacacagtactaagaaataaagacaggagacataggacttaacggtgatgggactcgtccactattctcattttaaggtaatgtaaccagaactcccctacccgtttgtgaaacctgagagaactataagatcaataatttataacgagtcgcattcaatctgttacttactctgaacaactacaaaagtaaagttaaacagaatattactagacacgagttgtacattttggttatctacattgtggaaaccttataaagactcatttgtaccccgtggttgagtttctcgttctccatttttacggatcacacctagttttagatgagatactgtcccttagagtacccgagacttcctaagaccagtgtatccctcatttatcgtctgagagttaagtctcagtctacactcaagtgtgcgttacaaaaccctgaagtaggacagaaaagggacgagaccctcagtattcttaattcaagattaggattaagacaacaatagatggactcactgtgattaatctatatattgaagagactccgagctgtaaatgtagatgtttatttcttccgatcttatgatttcggagaagataaagaaggttaataactaacatagccgagaatgagatatttaccaaagaagataaaatccctttaattaataaaacaagaataccacaacgacctggacaacgaaaagtaacgacattaatgaagagaaacaacttctggaaacggtctgctttacactacccacatattccgagaccgtaaaacgggtccagacatcgtgtatcttaaggtgattacccagacgacccgtagactctggtgtctcggtaaacagtattgtactgttaaggtcaacccgtccctatttacaatcgaaattgctaaaacctggtctcaaacagatctctctctcgtctcatgtttcggttttcgtagtagaaatctcgattcgtccgtactcaagtttagggttgggtcggtgaatgatctatacatcggtgtcggtggcggttcagagttaaatttacagtgaaagagtttgtccggaggatcccagagggtgcaaccgaatcaggtcttatgaccaaataggaatgccatattttaaataaggtagtaatacgtggtcataaattatttacgactccttacaccttgtttataaacaatttatttttcactgaattaggaagagacagagtcaggagtgaagtcacttcacccgttttcccatcttgttcaaaggacacgtttttcttagtccagtttcacgggatctttatcgtttgtgacagtgttgggatctatcgtactaatgttagactttatttgatcaagtttttcgtttagagtctgagttcaccccgaaaaagatcaaatcttgaacctcaatcttcttctttcttcccccgatttcacacgacgcacagatctacacggtccgtgacatgcattatcttacagtgtgtaaattataaacagattttcacactttcacacttaaaggtattctccctgtgtccaagaaccattttggttccaaacgagattgaaaagtgtgtgaaaccgtctgccaaaacggaaaaagaggattcaaccttgaaaactccggtaatgacggtcctcccttttcaatcactacgaatagatacaagtcttgatcttttaccggggaagaccaggggtcaaaccggggtaacaataagtgtacgacggatatttttctgttttggaggtcttccaccttttctacttatacgtcttacgatgtgtatctatgagtacatccactctaccgcttgtgtcgtctaaatccagatggttattctatgatggggtaaaccctactgtgtggaaggaatcttcactgtcaccgtcttgtatctgtttccctgattaattttcatacacccaagacgtctaacgtagacctcattctcaggtcactagatttaacatccggttccggagaacgaacgattgtaggagacagacggagtcaaaagaatggacgttttacctagtgacttgtagtgtaaagagaaataattaaataagtaagtgacttcttcgttcgacagtttttcgttgacgatgtatacagttctttctacggtctacgattttattttatgtttttaaactaatgatgtttaacgatggtagctcctcagtatcagattactttctctttttgtactctcacttattacttcagtcgtttttcaagttttctttttatttattttccgtatctataatttttacttcttcattttgatagaataagtctttcctatactaatacatgcctcttttagggtttcttagatgttgtagtctgagtagtcacttagatcgttctagtgacctatgtcaaatatatatttacaatagttattaacataaagacacggactgttgttttttaacttctgttgaaaattttgttgttacaaatattactgtggctttttatagtttaatcttcaagtacatttaacatcaaaggttctcgagggcgacctttaaccttcggtaacaactttatttaatttcttctaaattcgtttacctctctgaatggtaccaataccaagctttctgagatgtaacgattctacgttaaatgaggttttaacagatgtctaagttatgttaaagtcaatttcaaagactttgaaagtaaacaacaacaacaaaaaccttatctgttcgactaagacttcaaatatatgtttacgtttcctgcattttgtcgatttcttttaaacgtcttctttctttgattttcttaatgtgacagtctaaagctctggatgatgtttcgatgctaataattgtgtcacgtataaccatgttcttatccgtttatctgatttctttgtcttctgtctcaggtctttgacttgatgtgtatgtgctagtagactaaataatgtttccacggttccgttaactcatccttctcttgctacaagatgcatttaccgttataactcatagacataccattttttatttagaaccgatatacagtatattatacctgtttaattaatgtttacatcatatgtggtttacactttccattttgttttattgtacaatttttttcatatcatagaatggaaccctatcgtctataaagaatttgtcctgtgttcttcacttttccgttcggtgtcggagtgaaaacagaaggagtacggaagagaagatcacaccgagtcacgaatcacgtcctctttggtcattgggacttaacgtcgagaaggaagagtgatgtacttaagttaaaggagtagacagtttactcatatggttaagtatagagctttcgacaacgacactcttagtctattcgtattggagtgtcgaatacagataatcttgtcgtgaaccgtgtaccatttgtgaggtttcataaacaatttacttacttatctaattttccaccgtacaaaacatgatttgacaagttactatcacattttggtaaaccagtattacgcctttcccttcattccgccttaaggaaattagacacaaaatgcgtccaaggtttcctcgcaccacctctcttcctacgtctatcagacccactctcgatctccgacctcagtcgtccttcctgactccggcaaccacgaacccctcactcccgaggaaagacgagacaggatccgattcaaggggtgggtaaggaagaactctagatggagtttgtgtttagggagttaactggtgtcccccgcggggaagatacttaaaccgcgactatcgacactagacgggtcgtgtcaccccttttgtgttttaaatgtctagtccgtacaggcccgagtctaaggatgaggtcgtggaccaccggttccctggggttgacaatttatccgtaccactacggacgaaaggttcggacaaccctttctctctcccctcgcccctccttaccctctctctctctctgactcgttcgtacggttctgaattatatgaatataaatataattttctttatttatagtctactaatgttaaaccaacttgattctatgtgtcatcttataccttgattataggttatagtgtttcataagatcgctcggaaggatgtctttcttaacacccaccgacccctcatccgtaatcgatgatacactcacgtctcttatgagtcggaagaaggtctaccactcgatttcaagtttctagttcagtgcatgtgtggaagaaagagtagggtccaggatcagacgaacttaagtttaccggtaggtgtggaacggactttatgaacgttattaattctatgccgaaagacggacgaaccccaaaccaggtgttaagggaattctccggagtaaagttaatcctgagtgtgtagggaagttgtcattaaaacacagtccgaaccaatcgttgagttccgagttcgtatttaccctgtcttaagaaaaggaaaactttgagtggttatatcactaacatcgttgatcgatgtaacaaaaacaaaaaaaaaagggggagttaagattcgtgatacgtttccgaaatttcgtcaccagggttcggaaaaaccgtggtccctggtcaaaacaccttctgttaaaacacttttctgttttacaccttctggcacctgaccctaccaaacccctactaagttcgtgtaatgtaaacaacacgtgacacaaagataataataatgtaacataatatattactttattaatatgttgagtggtattacatcttagtcaccttcgggactcgaacaaaggacgttgatctgtgagggtagatccccactaccctctgccactgtccagtaatccgtaatctaagagtattcctcgcgtgttggatctagggagcgtacacgtcaagtactgtcccaaacacgacgatactcttaaattacggtgacgactagactgtcctccacctcgagtccgtcattccactcgttacccctcgtcgacatttattgcgactagagtgagtgggtgacgagtggaggacgacacaccgggtcaaggattgtccggtgttttaccatggacagacacaggggtcccaacccctggtgacggaatttccggaagtagagtaagtcaaaagtagttttaagacacaccatccatgagagtaatctgggtaaaatacccattccttgactccattttaaccaatatattgaacggattttattcagttcagagactactctcccggtcctaagttcaagttcgtcagactgaggttttagagtttcgtgaagacaccatcctttctctttacttaccttaccgtatctcagtagatttactgacgtcatccttccctcgtaaagggcacacgtcacaataaaaaaggcccgaaactttctatttatcctcgtacgtcaattttttctctcctcttccgtaagatccgtctttccggtcacgaatgtgtcttagagtcttaacattgtcaaggataatgtgggaccgtctcactacggttccgacaataacagttcgtgggaggacggagggtcaccccaactcttccccacttccctgtgaccgtcttcacttcgacccttcaaacgtgaacgatcaaccctgaacgtatcggtagaagagttacggtttctcctggagtcagagacacacgcgaaacaaaaaacaacaacaacaacaacaactaaacaccgggtccgatctcacgccaccacactagagacgagtgacgttggaggtagagggtccaagttccctaagaggacggaggtctgagggttcatcgaacctaatgtccgcgggcggtggtgtggacctattaaaaatatgaaaatcatccccacctcaaagtggcacaaccggtccgaccagacacacacgaaacctaaactctgtgagactactaaatctcaacttttaccctcatctaacccactaagagatcaatagtacaaatcagtttagtctaggcacgtaagttttagtattccgttcaaaaggacacaccgagtcattgtaggaatttctttatcaagactacaggtaggccacaaaaaagtctttctcgcagtcccaactgtcatcgacactacgaggtctacctcgacgcctattgtcgtatattcaaagtcccgtcaccaactccccgacaccctcccacccctcccttctacctactgaaaagagttggtagacataaactaaccttataacacactgaacactttatcttaatttctatactagaagaataccagaagagtgtcaaaagttccctaaaatcctcttttgcgaatcggtatgtctcgggttggaccattcaccgtcccgaccggtccagtcacgttgaagtttcagctacaacagtcacttacgaggtctacctaacgtctcttctggtttcaagtacagagccgtggaaagggttacatgtcccgaataacaaccctgtctcatcacggaccggatcttcaatttgtaagtaggtcgatcgataattccgaacttacggaagtttcttgtcgtacctaaaaagacacttagcactcgcaaaagcgttacgaattgtgccgtcgaccattactactaacgaggacaaagggaaacttaaagcacaagcaaatgaattgtcccgtaacgattagatcttcttccctcacccacttcttagggtaaacatttctcctatcgtccaattacttttcttcgtctccatacgcatccactatcacaaagatgttccgagccaagttaaccatactaaatttccgttcggaaccgaccgaccagtattattcccggtgtattacctcccctaaatgcaccgttaatggtaccaggaacgatcaccctatgttacaaaatcccgagggacctatgaattctaattacagacttagtcatcacaataacaacgttctagaatcacactaccctcggtacactccgtgcttaaaaatagggaatagtcttacattttatagagtatcagacgttcttgtggtcactgataccggacttcaacgggattctgtcaaatttgtaggacaactaacaaaacaaaaaaaaaggaaaaggaaccgttggtcttacgtacttactcagatcgcaatgaaaacaagtaggtccattatactaactttacccttaatatgtacaagttagtaaatctcttcttcctgatttttagtatctggatatcgtttaatttactaatatctcttagatggtacatttactgacgttaattcctgaagaagtacatggggcccggtctaagtgtcgtagaccctgtttgagaggtaccaaaaagggagccacataaataattcttactactaggacttgaagttcctctgaaccccttaaaaacctaaggacggtccatacatggaccggttctaattaaaccacttagtcttcaagggtccttggtatagtactcatgattctcttgtttaactaaatagatcatcatacaaagaggttgaatctatagacacgtttttttcacgtcgcctgtaccacgtgtaaggttcttcaagaggaggttccttcaccagttttatacattacgaataaataataggtaaaactctgggtttaataggtcagtcaccctagttatggaatgaggagaaggggtcttcggagtgtttatttcagaattgtggtagagttgtttttattctatccctggatctgtacctcttataccgacagagtacctaagattcgttagtccatctcataactctttacaataactttgtccttcaaggacgatttccacaaccaccctaaccctacggtcacgtctcactgtgtcataaacctgttcttgtgtattgtgctttcacagacttaggacaagaacagatattaccgtagaacggtaatttaggaa

SEQ ID NO: 3 - DNA, 465 bp, Homo sapiens
gaaaatcgggacagacaccgaagtcttattaaaggttgcgttggtaggtttaaaactgggtgtcgcacaatgtaaaccgtaacgccactgagtcaaggagtagaaatcacatgaggaagtagttccaaagattgtcgggtcaagacaggaccgaaaagaaggacgttgacaaaagtcgaacccactcagtgaaaagagagacctggaggtaaaagagtgggtgtagtgtcaggtcactcccgaagagaggtaggattttgaaagggggaccttgagttcagagagatacaacggacgttttaatcgaagtcagggtatatgaaccgggctaatgggtgtctttcatgtcgttcgtagtagtaggtgtatcccagaggttttaaccgaaaggaccttggtaagtgttccggtaaagtcagtttcggggttggaccattcaccgtcccgaccggtccagtcacgttg

SEQ ID NO: 4 - DNA, 8066 bp, Homo sapiens
agatttatacatatgtgtgtgtctgtgtttctaggttatcgtaaatggagttttgaaatcgatactttatcgttatctttgagtggtcaaatgtttgtccaagtgtaccgatttgataaaaacggggttatgtattagtttacttccgacacttggttttaaaccccatctcgtcaagagtaccgtcaaacgaaaaatttccggtatggaagggtctacggtttctcgtgatccaggtctatcgtggtgtctttttgtagtagatattggatgattagtccgggttgggacgaatcttgtcgtcgcatcctcagactgatgtaccttaaagtagaacggaagagtaagttgtcgtttgaggtctagggtttcttatgaccccggtccggttcacgtcaccgattgtggacgttagagtcgtgaaactctccgactacaccctcctggtgaactcaggttctcaatctctggtcggacccgttgtactacccttgaatagagaggtttttaatttttttttttttcgatccgtactaccgtacatggaaatgaggatcgatgaaccctccgactcgaccctcctagggaactcgggtcgtcaaggtccgatgtcactcggtactactgtgataacgtgaggtcggacccgttgtcgcattctaggacagagaccggttttttcccagaccgtggacgaatcctcccgaaggttttgaaaaagtcggagaaatccttcggaaggtagtaacacgacggaaggaggagacacgtcggagtcgtgagtgacaactcgggaagagatcctcaaacgttagatgcccctcactacccgtgtattcctttattaaagttacatcataccgtttacgactcgatctatttacgcgcttactgatacttcttgtctcctaaccccagtggattgagttgtactctgagtaccttcagaggactcctctttggagactcaggatctctcactcttaaccggtctttttaattcttccccgtcccttaaggtctctcttcattgtccatttgttttcgtttctccgtattctatcagacctcagaccagtttaatgttagtcaaccttcatcatctcttattttatgtttcacctctctcccctcttcatttcgacttatctatttgtcccagtcgaatgtctcccaggatacgtccgatttaaggtctacgacgatatttttatgtcctttcttttgagtactttataaaattctaaaaacaccttataaaattctcgaaaacacttgtagagtacttcgtgaggacacaaacctccgtcgtgaccgtcgtttagtttgtattattttccagacatgtagtttgtaactgtgtaaataagttgttcgtgtataactcgtggatgatacaccgtccttgagagaagtagtcgttcataaaaccgtgatttattttgtgtcttgtgtggcgggagaaactttactgttatttcttttattcacttaatatataatagagtcgtctataacgtaccatatacctttcgtatagtcccttcccccacatttcacagtactctccttaatgttataattatcctacaattctgtcgaggatgacttcggtacaaatttgtctgtgaacctcctctcctccctcaaccgattcaactataaaccccattccgtaaggtccttccccctagtcggtcaagtttcgggaccccccacccccgacacgaaccgtataaactcctcaccattcctccggtcacaccgaccttgtcttactagtttctttttccaccatcatttactccagtctatttgtcattctctgttccctaaaaatccagtagatcttaaatctaaaaaaggactctcccgtctcctcggtgctctttcgagactctactcctactctactagattaagtccaaaattgacctatcaagtctcgttctcacccccgtcccttggtcactcctctgacaccgttattagtgcttttcaccacgtcgccgaacctggtccctcaatcgtcaccttcgtctctcttcactgttgtgagacgtataccctttcccacccgtcctctcttgtcacgggttctactaggtcataaaaccggactcttcgacccctttttctttgttgttgttgttgtagtcaccttccccaaagtccctcaggtccacaagaccaacgtcgaaacaaaacggaatttttataaactcatgcattgatcattaccctaacgacccaacttaccattaaggcaaaaatcaggaaactctttaacggtgtcacgaaaggaatcgtttgattccgtccttgtcttttggtttacggtgtacaagagtgaacattcaccctcgatttactattcttgagtacttgtgtatctccccttgttctctatgactccggatggactcccacctccaaccctcctccctctcctagtcctttttattgattactcgtgatccgaattatggacccactactttcatagacatattgtttcaggacactgcactcaaagggatccattgtttgaacgtgtacacggggacttgaattttattttgatatatgtatatatatgtataatctttcttaatatgaaaactcaaaattatcgtgtaaaagacattctaaaacgttaaatttgaagtgatataaaatatatttgttaattctcaactcaactggaactataatgtataatgtctataaaataattgtagataattaaaaattaataaactaaaaaagttttaaagtttattatatggataaaaagtctaaagtccgtccggtaacttttcgaggatcaagattaatgacaaggacattacgaaatacttatattgtcaggccggaaaggagaatctcaaacgtcagattccatctctttatattattttcttttacgtacttaaaaattgattataccacacccaagatttcgagtctatttaataaagcaaatcaagagtgttgttgggagactacgtccgtgataataaagggggtaaaattattactcctttgacttcgtgtctctcgaaccaactgaacgggttataatggtgtgagacacaccgattcgaccctaaacttggttcttttgagagaagggtatccagcaactttttaatactttccaattcggtggagagacgaacacaacggataaaggtggtacactcaggttacacaccactgtctcttcccatctacaaaccgtagacacttaagacacctaacacacagtactaagaaataaagacaggagacataggacttaacggtgatgggactcgtccactattctcattttaaggtaatgtaaccagaactcccctacccgtttgtgaaacctgagagaactataagatcaataatttataacgagtcgcattcaatctgttacttactctgaacaactacaaaagtaaagttaaacagaatattactagacacgagttgtacattttggttatctacattgtggaaaccttataaagactcatttgtaccccgtggttgagtttctcgttctccatttttacggatcacacctagttttagatgagatactgtcccttagagtacccgagacttcctaagaccagtgtatccctcatttatcgtctgagagttaagtctcagtctacactcaagtgtgcgttacaaaaccctgaagtaggacagaaaagggacgagaccctcagtattcttaattcaagattaggattaagacaacaatagatggactcactgtgattaatctatatattgaagagactccgagctgtaaatgtagatgtttatttcttccgatcttatgatttcggagaagataaagaaggttaataactaacatagccgagaatgagatatttaccaaagaagataaaatccctttaattaataaaacaagaataccacaacgacctggacaacgaaaagtaacgacattaatgaagagaaacaacttctggaaacggtctgctttacactacccacatattccgagaccgtaaaacgggtccagacatcgtgtatcttaaggtgattacccagacgacccgtagactctggtgtctcggtaaacagtattgtactgttaaggtcaacccgtccctatttacaatcgaaattgctaaaacctggtctcaaacagatctctctctcgtctcatgtttcggttttcgtagtagaaatctcgattcgtccgtactcaagtttagggttgggtcggtgaatgatctatacatcggtgtcggtggcggttcagagttaaatttacagtgaaagagtttgtccggaggatcccagagggtgcaaccgaatcaggtcttatgaccaaataggaatgccatattttaaataaggtagtaatacgtggtcataaattatttacgactccttacaccttgtttataaacaatttatttttcactgaattaggaagagacagagtcaggagtgaagtcacttcacccgttttcccatcttgttcaaaggacacgtttttcttagtccagtttcacgggatctttatcgtttgtgacagtgttgggatctatcgtactaatgttagactttatttgatcaagtttttcgtttagagtctgagttcaccccgaaaaagatcaaatcttgaacctcaatcttcttctttcttcccccgatttcacacgacgcacagatctacacggtccgtgacatgcattatcttacagtgtgtaaattataaacagattttcacactttcacacttaaaggtattctccctgtgtccaagaaccattttggttccaaacgagattgaaaagtgtgtgaaaccgtctgccaaaacggaaaaagaggattcaaccttgaaaactccggtaatgacggtcctcccttttcaatcactacgaatagatacaagtcttgatcttttaccggggaagaccaggggtcaaaccggggtaacaataagtgtacgacggatatttttctgttttggaggtcttccaccttttctacttatacgtcttacgatgtgtatctatgagtacatccactctaccgcttgtgtcgtctaaatccagatggttattctatgatggggtaaaccctactgtgtggaaggaatcttcactgtcaccgtcttgtatctgtttccctgattaattttcatacacccaagacgtctaacgtagacctcattctcaggtcactagatttaacatccggttccggagaacgaacgattgtaggagacagacggagtcaaaagaatggacgttttacctagtgacttgtagtgtaaagagaaataattaaataagtaagtgacttcttcgttcgacagtttttcgttgacgatgtatacagttctttctacggtctacgattttattttatgtttttaaactaatgatgtttaacgatggtagctcctcagtatcagattactttctctttttgtactctcacttattacttcagtcgtttttcaagttttctttttatttattttccgtatctataatttttacttcttcattttgatagaataagtctttcctatactaatacatgcctcttttagggtttcttagatgttgtagtctgagtagtcacttagatcgttctagtgacctatgtcaaatatatatttacaatagttattaacataaagacacggactgttgttttttaacttctgttgaaaattttgttgttacaaatattactgtggctttttatagtttaatcttcaagtacatttaacatcaaaggttctcgagggcgacctttaaccttcggtaacaactttatttaatttcttctaaattcgtttacctctctgaatggtaccaataccaagctttctgagatgtaacgattctacgttaaatgaggttttaacagatgtctaagttatgttaaagtcaatttcaaagactttgaaagtaaacaacaacaacaaaaaccttatctgttcgactaagacttcaaatatatgtttacgtttcctgcattttgtcgatttcttttaaacgtcttctttctttgattttcttaatgtgacagtctaaagctctggatgatgtttcgatgctaataattgtgtcacgtataaccatgttcttatccgtttatctgatttctttgtcttctgtctcaggtctttgacttgatgtgtatgtgctagtagactaaataatgtttccacggttccgttaactcatccttctcttgctacaagatgcatttaccgttataactcatagacataccattttttatttagaaccgatatacagtatattatacctgtttaattaatgtttacatcatatgtggtttacactttccattttgttttattgtacaatttttttcatatcatagaatggaaccctatcgtctataaagaatttgtcctgtgttcttcacttttccgttcggtgtcgggttggaccattcaccgtcccgaccggtccagtcacgttgaagtttcagctacaacagtcacttacgaggtctacctaacgtctcttctggtttcaagtacagagccgtggaaagggttacatgtcccgaataacaaccctgtctcatcacggaccggatcttcaatttgtaagtaggtcgatcgataattccgaacttacggaagtttcttgtcgtacctaaaaagacacttagcactcgcaaaagcgttacgaattgtgccgtcgaccattactactaacgaggacaaagggaaacttaaagcacaagcaaatgaattgtcccgtaacgattagatcttcttccctcacccacttcttagggtaaacatttctcctatcgtccaattacttttcttcgtctccatacgcatccactatcacaaagatgttccgagccaagttaccatactaaatttccgttcggaaccgaccgaccagtattattcccggtgtattacctcccctaaatgcaccgttaatggtaccaggaacgatcaccctatgttacaaaatcccgagggacctatgaattctaattacagacttagtcatcacaataacaacgttctagaatcacactaccctcggtacactccgtgcttaaaaatagggaatagtcttacattttatagagtatcagacgttcttgtggtcactgataccggacttcaacgggattctgtcaaatttgtaggacaactaacaaaacaaaaaaaaggaaaaggaaccgttggtcttacgtacttactcagatcgcaatgaaaacaagtaggtccattatactaactttacccttaatatgtacaagttagtaaatctcttcttcctgatttttagtatctggatatcgtttaatttactaatatctcttagatggtacatttactgacgttaattcctgaagaagtacatggggcccggtctaagtgtcgtagaccctgtttgagaggtaccaaaaagggagccacataaataattcttactactaggacttgaagttcctctgaaccccttaaaaacctaaggacggtccatacatggaccggttctaattaaaccacttagtcttcaagggtccttggtatagtactcatgattctcttgtttaactaaatagatcatcatacaaagaggttgaatctatagacacgtttttttcacgtcgcctgtaccacgtgtaaggttcttcaagaggaggttccttcaccagttttatacattacgaataaataataggtaaaactctgggtttaataggtcagtcaccctagttatggaatgaggagaaggggtcttcggagtgtttatttcagaattgtggtagagttgtttttattctatccctggatctgtacctcttataccgacagagtacctaagattcgttagtccatctcataactctttacaataactttgtccttcaaggacgatttccacaaccaccctaaccctacggtcacgtctcactgtgtcataaacctgttcttgtgtattgtgctttcacagacttaggacaagaacagatattaccgtagaacggtaatttaggaa

SEQ ID NO: 5 - DNA, 1824 bp, Homo sapiens
ttctatcactcaccgttttggatcgtacttcgggtctcatacaccgagacgcaatcataaagagtgtcgggtgacattactgacagtccaacgaaaattctaatactttcaggatataacttaacagtaagcttaactctggaacttcagacttctgccttaatgaacccttcttcgtagtgtcatagaatcttctcacagggaggtacttcgtctaaaccccagagtaaggcaaagacatgaatgtcattacctggtacaatccgttcagtaaattgtgtaaacctggggtcgaaggtttagatatgttaccttccatattaacctctctcatatttcggaaatcacgggtgaaatgaactctctaaaagtctcgtcagttactctgaaatctttattttcacttgaattttgtatttcacgaaatatttggggtcgtaacggacttcgggactctaacgaactaccgggtaacgcatataagtgtccgtgacggggttgaccgggaatgatgttgagatctttactgtccgtaagtaagaaggttaggtgtctactccgttgatgcttcacaataaaaattggggagtaaaaaattcctctttttgactcgaactcgtgtaattttttacaccgggtctcagttataccatatacaactggaaccttaagctcttttcagaagacagtgttctcgtcttcggtgtttgagtttatgaaaatcccaatacaatggttaacaccttgtgtacacgtactttactcgactcattctacggtttactggaccataacctctccgttatccctcaccaccccggacatcgtttgatctctctcgtaccgagtcaattttctctcaccgtcgttgagttgaggtcggttaacaacggtatgttataattcgggtccctaaagtcttgaagatcgatctttttatctccgatctatacatataaggacaagttttaacggagttaatcttctataatcgttcattaagtttacgttatgtgaaaacataatagtgatatgaccaggtggattattcccctgtcaaacgaaggacgagagtgtttcacaaagtctgattcaatactggtgaattcatacgtttctgttttgtcacatagtcattacgtcactaacactcgtacatgaagtctttgtttactagacccaagtttaggaccacaactgtaattcatcaaattattggagcccgttcagtgaactgaagagatatggagtcaaagggatagacattttaccttcattattctcatgaatgaggaaagtcaccaacactgatagtttacttaactgtatccattttgttaatcttgtcaaggactgtgtgccattctcagtacatttatagttacgaatactttcgagagtagggtcctattcgtagaggatcttttgtagaagcaggtacatggtctaattagtataaataagacgtcaactataaatacggtgtacaagaaagacccatctcttcggacttcaataagacaaataggactggaaccttttctgtttcgtcgagtacaggggtccctagatttttaaagtgacccttactagtgggtcacagaggttttggagtcggtcgtaaagagataagtgtcgacgtgacttctcgaaggaaggaccgaacacagaggttttcccctatgctaccgttccaacaaataatgagagtccgactacaccggcccctctacaccttaacacatcttaccttacgctaccttatactttaccacaccttatgtggttggaccattcaccgtcccgaccggtccagtcacgttg

SEQ ID NO: 6 - DNA, 11053 bp, Homo sapiens
actgtttatttagtttaaaccctacggagttgtgttctttataaaaatacatagtaatacattgtcaggtccctccgacttttatctcacatacaacgtccattctttaaaacgagacgtcagtaagtccttaacttcgactatcactaagacggtagaacttgtacaccgtagcgacagacagacctcccacggtagtgtcagtcaaacctgtcgtggaacttacgatagtcccttcgatctcacaagaggacaagaaacgacaggaacggtcacagaagaggacttgagtgtagtcttcgtacgtcattcgtccaccatggtcgtcccaagattgggtccgtgaggttaagattccagttgaaacaatcacaatagattttttcttttcgttattatttaataggtgttcttttaaaatgttgagttcaaaaagtatgagaaatttttccgtaaaaaagtgtacatgagagtacaagatactaatctggattagtaacagtgaagtgccgatctctttgattctggtcttctcgaaggtctagaactgatcgtggtgagttactcaccctactggtcttgggacatgactagtacgtttgaagtggtgtattgtcgaacactataactcactcaacaaagtggatatgctggggagatttggttaaataattagatcttttacccttattatcgttaaagatacattattcaacaacctcgtgttctatttcaatatacatattttgtaaatcgtgtcaaggaccacgtattgtccagacatcatttataaacaacattaatcgtcgttttagtagagggagtaatgacgtcaactaaaaggaaataataacctttctttaaagagttgactcaaagtcaacttatgtcataatctaataaggaattgactcaaagtcgtaaaatttacatatgagggatgagttttgatggatgatttagtgcggacattaaggtcgtgagaccgtccggttccgcccacctagtactccagtcctctagttctggtaggaccgattgtgctactttggggtagagatgattttttacgtttttttaatcggtccgcaccaccgaccgtggacatcagggtcgatgaaccctccgactccgtcctcttaccacacttgggccctccgtctcgaacgtcacccggctctagcacggtgacgtggtgtcggacccgctgtctcactctgaggcagagtttttgtttgtttttttgtgtttttagatggatgatttttcttcaagaagttacgaatctgaaactcgtttctttttcagacgagattgtccttcgaccactatatctttccatttcaaagtgaagtgtccgtgaaactaaagggaagctccacctatgacttactaaacacacacgcgtgtaaaaagatacgtaataagttttaattttaaggaatctcctttggtgactttcggttagtaaatgttttgaaatttttactgtagaacttctcaagaaaccacgagtaagtagtttgaatcgttactaaattgacattaagaaataagtctaagtagagggtgttttatttttacggtatttcgaaatgtcatgacataggattacttatctctttgatttctttttcattctactcgttcactctccttttgggcttttactcggacaggaccgtacaaagatttttctttctttgtttgtttgttcgtcggggaggagagtcgagaaccctttctttataacttagaactgttatagacgtgaagtatcaactaagtatcgtactggatagagtttgttaaattctaagtttacttcaaacgttaattagaaagctatagtgaaacgttttgtaagagtattggaataggtcgggaaaatgtttagttaggacactccacttgtagtgacacaagggtaaaatgtctctttccgtgactcggtgtctctccaatatatgagtactagttattcgaccattctgattcttggtccttactatgacagaaggaagaggtttataggacaagaaataatactcatggatttgtcataatttttaattaatgtcgagttgttatcattcatttacaggagtacactttaggtggcaaattttgaattccaatagataaatagtttatttaatttaggatgagtgaattgttataagtaactcgagtaagacatttgttggtaatccggtccccgtctatactttatactccgagttagacactagtgtctctactttatatgttaaatctctctctttctattcgtactactgtttatttattacatacttttaatcggtaatagaatccggttgaaaaagattcgacattcgacagacggatgaagacggtccacaatcattaacaaaatttttcacccccttcttctcatgaagtaccacccttctataagtaactcctgtattcgtagaaggagaatctttaattgttacgtgtcaccggataacgttcaaaactttcgggacgtttgttattttcggactaatcaaaaataacttagtcatagaggatttgtgaaaaagtactttgttccaatgagtgtttagaacagctccttgattacaggatcctttcaccaaaagttcgaactcgtacatgtattcatagtaacctttccaacgtttttatgtttacacacccgaggtgaggtctttaagactaacttcaccagagtagacagtagactcttgaacgtaaaaacagtctaaggatcgactagactacaaagtcctgactcttgaattaaactcatcatagagatgtcttgtcaaaaattttacaagaggacctcatcctactaatatgaattgtttttacattatgtgagtccactacctgtgggaatcataggactaacctagtgatgtgtaatatatgtacattgtgtaaaagagttcatggggtatttaaacgtgtttatttatttatttattttaatatgaaaagagtttatttttttattttatttacaaggagaacttaccatcttagaaacaaaaaaacactattagtatttatgtatatttataagagtagtaatgtacgtacatcaatggaaggaaatgtactacgtggtctttcttatgggtgagattcttcctttcttacttctcttcttccgtaacaaattttctggataataatcttattcagtttaagatacagatggtaataattcgacaaactgaaactcgtccctaaccttccgtaaaatttaactccacctctatacgtgtttcggtgcaccctttacagtacacagggacgtatttctcttgttcgataaaacgaaccaacctctactcctctgtctccgacatgtattcttacacaagttaaatttcgttgttttatatagctggtttgatgaaactcgttagttcccctatataaccgagtgtagtgactttatatatgaccgtgtcgtctaaaggtcaatccagactagacgatcgagacaggggaggtcttatgtccgaggtccgtccgtccttccttctcctgtagtcaagagaaccacagatcgtgcgacggacataattccatccaggagttatttaagtacaacatcctttacttacgtacaagagtttctacgccaatgaaagtcatagtgacgaaaggagtaccaaaggtgaagttataatcagattgaacggaatccctgggttctaccgacgataagtgaagttaatcgatttgtgaagagaaaagtaccgacactctctgatcgatggagaaggtatttacttaaaagagaagaaagacccgtgttatcagagataaagggtcggagaaaatgttaatccacataggtacgttgagtcaagatcggttaccgcacactcatcatcactataggtggtgaacgtctggatgtgtatttccgagggtctgtgtagaagacacgagaaatgaccttgtgaacgaactaaggttatttatgtcgttggaatcgtcgatgtataacgtcaaccgtctcgaaagtacaaagtcgaagaagtataaaaaatcaaaacaacagtgacaaccaaaaaaaaaattaactaagtcctctactggattattttttaacttctttttatttcgtaaaacaagacctaaagagtaatccttgtactccaaatgagataacgttgaccgaatcaagtatactagtaggggactccactccctttttctacgcacttaactaattcggttccagtgtaccagctttacatcttaacccaaaactccagtcaaagggatttagtgggtctataggttcacctttagtccgaggtaactgttttcccttgtcaagaatctttacgttgatgtttacaggttagggtcaaccgttcaagcttcgttccttcccgaaaggtaatttcttacacctacgatggaccacccgttgacctccggtgaccgtatataaaaaaaaccccccccaaagtatttgataaccaaaaaaattaataataatatgaaattcaaaatcccatgtacacgtgttacacgtccaatcaatgtatacatatgcacacggtacgaccacacgacgtgggtaattgagtagtaaatcgtaatccatatagaggattacgatagggaggggggaggggggtggggtgttgtcaggggtctcacactacaaggggaaggacacaggtacacaaaagtaacaagtcaagggtggatactcactcttgtacgccacaaaccaaaaacaggaacgctatcaaatgactcttactactaaaggttaaagtaggtacagggatgtttcctgtacttgagtagtaaaaaataccgacgtatcataaggtaccacatatacacggtgtaagagaattaggtcagatagtaacaacctgtaaaccgaaccaaggttcagaaacgataacacttatcacggtgttatttgtatgcatacgtacacagaaatatcgtcgtactaaatatcaggaaacccatatatgggtcattaccctaccgacccagtttaccataaagatcaagatctagggactccttagcggtgtgactgaaggtgttaccaacttgatcaaatgtcagggtgattgtcacattttcacaaggataaagaggtgtaggagagctcgtggacaacaaaggactgaaaaattactaacggtaagattgaccacactctaccatagagtaacaccaaaactaaacgtaaagagactaccggtcactactactcgtaaaaaagtacacaaaaaaccgacgtatttacagaagaaaactcttcacagacaagtacaggaaacgggtgaaaaactaccccaacaaacaaaaaaagaacatttaaacaaactcaagtaacatctaagacctataatcgggaaacagtctactcatccaacacttttaaaagagggtaaaacatccaacggacaagtgagactaccatcaaagaaaacgacacgtcttcgagaagtcaaattaatctaggggaaacagttaaaacagaaaacaacggtaacgaaaaccacaaaatctgtacttcaggaacgggtacggatacaggacttaccattacggatccaaaagaagatcccaaaaataccaaaatccagattgtaaattcagaaattaggtagaacttaattaaaaacatattccacattccttccctaggtcaaagtcgaaagaggtataccgatcggtcaaaagggtcgtggtaaataatttatcccttaggaaaggggtaacgaacaaaaagagtccaaacagtttctagtctctcaacatctatacaccgcaataaagactcccgagacaagacaaggtaactagatatagagacaaaaccatggtcatggtacgacaaacccaatgacatcggaacatcatatcaaacttcagtccatcacactacggaggtcgaaacaagaaaaccgaatcctaactgaaccactacgcccgagaaaaaaccacggtatacttgaaatttcgtcaaaaaaggttaagacacttctttcagtaaccatcgaactacccctaccgtaacttagatatttaatggaacccgtcataccggtaaaagtgctataactaagaaggatgggtactcgtaccttacaagaaggtaaacaaacataggagaaaataaagtaactcgtcaccaaacatcaagaggaacttctcaaggaagtacagggaacattcaacctaaggatccataaaataagagaaacttcgttaacacttaccctcaagtgagtactaaaccgagagacaaacagacaacaaccacatattcttacgaagactaaaaacatgtaactaaaaatataggactctgaaacgacttcaacgaatagtcgaattcctctaaaacccgactctgttaccccaaaagatctatatgtacagtagacgtttgtccctgttaaactaaaggagaaaaggattaacttatgggaaataaaggaagaggacggattaacgggaccggtcttgaaggttgtggtacaacttatcctcaccactctctcccgtagggacagaacacggtcaaaagtttcccttacgaaggtcaaaaacgggtaagtcatactataaccgacacccaaaaagtatctattgagaataataaaactctatgcagggtagttatgaattaaataactctcaaaaaccgtacttctcaacaacttaaaacagtttccggaaaagacgtagataactctattagtacaccaaaaacagaaaccaagacaaatatacgacctaatgtaaataactaaacgaatataacttggtcggaacgtagggtccctacttcgggtgaactagtaccacctattcgaaaaactacacgacgacctaaaccaaactggtgaccgtataaaattcgtaccctcattgtgacagtccaaaaaatttaatgttttacgaaatcgtatctcttttaatatttcttgttatattcattgtctatacgtgagtgataggacgaattagtttacagtgtgaaacggttcgaactaagtttaaaaaatttcgtttctttgtaatgtctataccgacgttgtaggatacacggggtggcgactatgtatggagagaagggttcccattggtgaaagactgaaactatgaatagtaagggtccgtactaatttacgataacgacttaaacgtatatatgtatttattatatatgtcaacaaacgtacaagattttgaaacgtaatttattatagtttattaatttttaaaagtgtttaacgtaaaaattgagtcagaaaatattctaacggttattactatagagaagtctagtaagtaaaactgataatataataaaaagtaacatactgatacggtaccgagtgaataggtaagacaataactatttgtaaacacaacaaaggtgttaaaacgataattttattaccgtaacacttgtaagaacacacatatagtgacacatgtgtacgatctcaaagagattacataataccacatataacgacccggtttccgatacattcagaagttgaagggatctacagtatggttgagtatgtatatactggtcacactcgtaagagtcacgagatgtaacaggtctaagatgtacttcgtgaccaccggataaccagtccaactgactataatcttccaataacggtttcagatacactctctctgactcccagactttatggatctacattccctatatttcactctctcctttcttcaattgtataaatcctcgttttaggtgtactgaaacactaactaatacctcttttattcctcttcttcccttgtccttctgagagttcagaggtctaacttgtgttctccttcgaatacacggcactctgactactgtttaaggaaaacttgtatcacggaaactcccgaaccatcattttttctttcgtgataggtagtccgtaaacctataaatccagaccttctgacttttctctagttttgtcttttatgtttaatatcttagtagctctacccattttagtcttctcaacctagttcttttcatggatcttagtcatctcttcactcaattcttttatagagaccctttgtaattataaatttccatatattttccttctcttctgacacctcttctgtctctgacttcttcctctgttttacacagtatgacatcatcggtctccttatctcgaagtttcttactcaccagttggtgtaatttgtgtcgatcttttggttcttccatttctttacttttaatttgtaattgtatgttacttcaataactcaggtacaattttaccaaagttaccttatcgtagttacctttattaacgttaatcattttcttaaaatctttttcttttttaattatgtcgattgaaagagtttaatttaaaaaacttttattttgtcactctaccttaagctcacgttctacaaacaacttttagttgtgtgtactttcctttctctcacttggatttttttaaccgaggtctcagataattacatttctgatacaatataacagagagatagaaatccctttgtatatgggttaagtagaacacagtggtcttagtctaagtagtttgggtaagacctggtgagactagtgatcaaagtgggagtgtcagtatcatttctttgatttcgttttctgatgttctcgtttcctgtctttccctttacaataaaagaggggagtggaaacgggagaaactaaaagaggtaacaacgattttccttgtgaatcttttgatactttctttgaagacggacatttacgtcgaggtactaatacttaagacttaggaacattgtcttcttggttatcctgactaggtactgaagataatcatctctgacccttccatccactgaaatcgagtggttcggactagtgtcgttttatcttttactagtgtcacaggggaaaaataggaccccattgttacttgtaagtcaccctcggttgatgacataatttcaggacccacgtcgaggaccgtgtactgtaccgggtgttccatcatcaagactcatgggaacggatagtcaccacgaccccgctcttccctcccgtcggacgagtgatccctctcgtccttactccgatccttcatgtccctggaccgtttctacagaggacaaactctctctgaagtcaattacaagtcagttgaaggacaccacgattcttcactttcaacttgaactgatagttccttgtctccgtccaacaatcgacccggggaccctccttcagttgttcgaggtggtgtagactgttgtggatgacgaacgtcgggaagggggtccagtccgtcgacgtgtggagtacgaaggttgactcccccttacttacccatggttctcatccactcagatgaagaaagggtccccactcatcgcccacttctttagtcgtacatcacctgtaaatgtacacggcctatggagtatatacgtcacaccatagtaataggagtgacacgtctacttctgtgactccgagtccctgaacaagttctgtgtgtagaccagttatccctcggtcctaagttttagtgcagtcagatcatgagttcaggagacaagaaaggtgctgatgtaatctacatagggatctatcagatccacattgtcgtactcagagggtactttccttcacccccgagaaccttgtatggagaaatccttcggaaggtagtaacacgacggaaggaggagacacgtcggagtcgtgagtgacaactcgggaagagatcctcaaacgttagaaccctatcgtctataaagaatttgtcctgtgttcttcacttttccgttcggtgtcgggttggaccattcaccgtcccgaccggtccagtcacgttgaagttcagctacaacagtcacttacgaggtctacctaacgtctcttctggtttcaagtacagagccgtggaaagggttacatgtcccgaataacaaccctgtctcatcacggaccggactgaaagcggttttcgtacgtgtcttgcaccttgaaccggaggacttttccgcacagaagtcgaatccaataaggaaagagctacgagtggtactacagtccgaggatcatcctctcggtaattattgaagccactgaaccgtaaactacccgttagaaccggtaggatttcgtaaggtacggtagtctatatgggacgtaacggtactcgaaatagtaaccgaaaatcttgtagtaggagggtgaaacttatttaccagatcgtctgttatgtcaggaacacggtccgttgtaagacctacgaaatacatgtaatcgagtaacttagtaaagttaagttagtaagttgcgtccccaaacttagaatcgacaaactccagtaacaggtacgtgagtggatattgtaacaagacagagaaagacgtttacattctatttttataatggaagtaagatcttttgtggggaaacatcttatccaaatatggaagtccgtacacctgaaaggttaggtttgaggtcctcatctgtctatgggtggtcctgatccgttacgtccttttagagtccgaagtcgatcctgacaaagtatgttaaaggacgtaccggtccttgttcccacttccgtacgtgagacactcgtcgggtaaacacctgtcacccagtaccctgacttccttggtacaatgtgtacggactcaaaagaaaggttcgagtctttggtatagcttgtggggagggaacccctcttcactcactcgtccacctctctgctatcattacaatcataccaccttgaagaaggggtatctacctttgtgactcccgattcttcttcccggagaggaggttgtacacaatagatcgttccgaccaagataaattcttactatatatcagatcacattatcttatgttatacggatcgagattttaatacaacctttttttagttgtaatgctacacgatataagtcagttactcatttataaagacacggacggtgtacg

SEQ ID NO: 7 - DNA, 1166 bp, Homo sapiens
cgtcgttacggatctttactaccaagaagtttaggttcactattgggtatcattgattgagtaatcgaatcaagacggcatttcagtcttgtttcgttcctctttgtcttggagacgtcacttacctccttaaagactcccagtgaactttcgtctttgagttctcgggttggaccattcaccgtcccgaccggtccagtcacgttgaagttcagctacaacagtcacttacgaggtctacctaacgtctcttctggtttcaagtacagagccgtggaaagggttacatgtcccgaataacaaccctgtctcatcacggaccggactgaaagcggttttcgtacgtgtcttgcaccttgaaccggaggacttttccgcacagaagtcgaatccaataaggaaagagctacgagtggtactacagtccgaggatcatcctctcggtaattattgaagccactgaaccgtaaactacccgttagaaccggtaggatttcgtaaggtacggtagtctatatgggacgtaacggtactcgaaatagtaaccgaaaatcttgtagtaggagggtgaaacttatttaccagatcgtctgttatgtcaggatattgtaacaagacagagaaagacgtttacattctatttttataatggaagtaagatcttttgtggggaaacatcttatccaaatatggaagtccgtacacctgaaaggttaggtttgaggtcctcatctgtctatgggtggtcctgatccgttacgtccttttagagtccgaagtcgatcctgacaaagtatgttaaaggacgtaccggtccttgttcccacttccgtacgtgagacactcgtcgggtaaacacctgtcacccagtaccctgacttccttggtacaatgtgtacggactcaaaagaaaggttcgagtctttggtatagcttgtggggagggaacccctcttcactcactcgtccacctctctgctatcattacaatcataccaccttgaagaaggggtatctacctttgtgactcccgattcttcttcccggagaggaggttgtacacaatagatcgttccgaccaagataaattcttactatatatcagatcacattatcttatgttatacggatcgagattttaatacaacctttttttagttgtaatg

SEQ ID NO: 8 - DNA, 4103 bp, Homo sapiens
tgaaaacagaaggagtacggaagagaagatcacaccgagtcacgaatcacgtcctctttggtcattgggacttaacgtcgagaaggaaagtgatgtacttaagttaaaggagtagacagtttactcatatggttaagtatagagctttcgacaacgacactcttagtctattcgtattggagtgtcgaatacagataatcttgtcgtgaaccgtgtaccatttgtgaggtttcataaacaatttacttacttatctaattttccaccgtacaaaacatgatttgacaagttactatcacattttggtaaaccagtattacgcctttcccttcattccgccttaaggaaattagacacaaaatgcgtccaaggtttcctcgcaccacctctcttcctacgtctatcagacccactctcgatctccgacctcagtcgtccttcctgactccggcaaccacgaacccctcactcccgaggaaagacgagacaggatccgattcaaggggtgggtaaggaagaactctagatggagtttgtgtttagggagttaactggtgtcccccgcggggaagatacttaaaccgcgactatcgacactagacgggtcgtgtcaccccttttgtgttttaaatgtctagtccgtacaggcccgagtctaaggatgaggtcgtggaccaccggttccctggggttgacaatttatccgtaccactacggacgaaaggttcggacaaccctttctctctcccctcgcccctccttaccctctctctctctctgactcgttcgtacggttctgaattatatgaatataaatataattttctttatttatagtctactaatgttaaaccaacttgattctatgtgtcatcttataccttgattataggttatagtgtttcataagatcgctcggaaggatgtctttcttaacacccaccgacccctcatccgtaatcgatgatacactcacgtctcttatgagtcggaagaaggtctaccactcgatttcaagtttctagttcagtgcatgtgtggaagaaagagtagggtccaggatcagacgaacttaagtttaccggtaggtgtggaacggactttatgaacgttattaattctatgccgaaagacggacgaaccccaaaccaggtgttaagggaattctccggagtaaagttaatcctgagtgtgtagggaagttgtcattaaaacacagtccgaaccaatcgttgagttccgagttcgtatttaccctgtcttaagaaaaggaaaactttgagtggttatatcactaacatcgttgatcgatgtaacaaaaacaaaaaaaaaagggggagttaagattcgtgatacgtttccgaaatttcgtcaccagggttcggaaaaaccgtggtccctggtcaaaacaccttctgttaaaacacttttctgttttacaccttctggcacctgaccctaccaaacccctactaagttcgtgtaatgtaaacaacacgtgacacaaagataataataatgtaacataatatattactttattaatatgttgagtggtattacatcttagtcaccttcgggactcgaacaaaggacgttgatctgtgagggtagatccccactaccctctgccactgtccagtaatccgtaatctaagagtattcctcgcgtgttggatctagggagcgtacacgtcaagtactgtcccaaacacgacgatactcttaaattacggtgacgactagactgtcctccacctcgagtccgtcattccactcgttacccctcgtcgacatttattgcgactagagtgagtgggtgacgagtggaggacgacacaccgggtcaaggattgtccggtgttttaccatggacagacacaggggtcccaacccctggtgacggaatttccggaagtagagtaagtcaaaagtagttttaagacacaccatccatgagagtaatctgggtaaaatacccattccttgactccattttaaccaatatattgaacggattttattcagttcagagactactctcccggtcctaagttcaagttcgtcagactgaggttttagagtttcgtgaagacaccatcctttctctttacttaccttaccgtatctcagtagatttactgacgtcatccttccctcgtaaagggcacacgtcacaataaaaaaggcccgaaactttctatttatcctcgtacgtcaattttttctctcctcttccgtaagatccgtctttccggtcacgaatgtgtcttagagtcttaacattgtcaaggataatgtgggaccgtctcactacggttccgacaataacagttcgtgggaggacggagggtcaccccaactcttccccacttccctgtgaccgtcttcacttcgacccttcaaacgtgaacgatcaaccctgaacgtatcggtagaagagttacggtttctcctggagtcagagacacacgcgaaacaaaaaacaacaacaacaacaacaactaaacaccgggtccgatctcacgccaccacactagagacgagtgacgttggaggtagagggtccaagttccctaagaggacggaggtctgagggttcatcgaacctaatgtccgcgggcggtggtgtggacctattaaaaatatgaaaatcatccccacctcaaagtggcacaaccggtccgaccagacacacacgaaacctaaactctgtgagactactaaatctcaacttttaccctcatctaacccactaagagatcaatagtacaaatcagtttagtctaggcacgtaagttttagtattccgttcaaaaggacacaccgagtcattgtaggaatttctttatcaagactacaggtaggccacaaaaaagtctttctcgcagtcccaactgtcatcgacactacgaggtctacctcgacgcctattgtcgtatattcaaagtcccgtcaccaactccccgacaccctcccacccctcccttctacctactgaaaagagttggtagacataaactaaccttataacacactgaacactttatcttaatttctatactagaagaataccagaagagtgtcaaaagttccctaaaatcctcttttgcgaatcggtatgtctcggttggaccattcaccgtcccgaccggtccagtcacgttgaagttcagctacaacagtcacttacgaggtctacctaacgtctcttctggtttcaagtacagagccgtggaaagggttacatgtcccgaataacaaccctgtctcatcacggaccggactgaaagcggttttcgtacgtgtcttgcaccttgaaccggaggacttttccgcacagaagtcgaatccaataaggaaagagctacgagtggtactacagtccgaggatcatcctctcggtaattattgacggatagagtggtaatctgacacatgaagatcttccgtctttagaaaaagattactaaagaataaagggtcttggatattgtaacaagacagagaaagacgtttacattctatttttataatggaagtaagatcttttgtggggaaacatcttatccaaatatggaagtccgtacacctgaaaggttaggtttgaggtcctcatctgtctatgggtggtcctgatccgttacgtccttttagagtccgaagtcgatcctgacaaagtatgttaaaggacgtaccggtccttgttcccacttccgtacgtgagacactcgtcgggtaaacacctgtcacccagtaccctgacttccttggtacaatgtgtacggactcaaaagaaaggttcgagtctttggtatagcttgtggggagggaacccctcttcactcactcgtccacctctctgctatcattacaatcataccaccttgaagaaggggtatctacctttgtgactcccgattcttcttcccggagaggaggttgtacacaatagatcgttccgaccaagataaattcttactatatatcagatcacattatcttatgttatacggatcgagattttaatacaacctttttttagttgtaatgctacacgatataagtcagttactcatttataaagacacggacggtgtacg

SEQ ID NO: 9 - DNA, 2612 bp, Homo sapiens
tcatcattaccagctgccgtgttaagcattgcgaaaacgctcacgattcacagaaaaatccatgctgttctttgaaggcattcaagccttaatagctagctggatgaatgtttaacttctaggccaggcactactctgtcccaacaataagccctgtacattgggaaaggtgccgagacatgaactttggtcttctctgcaatccatctggagcattcactgacaacatcgactttgaagttgcactgacctggccagccctgccacttaccaggttggctctgtatggctaagcgttttctcctaaaatcccttgaaaactgtgagaagaccataagaagatcatatctttaattctatttcacaagtcacacaatattccaatcaaatacagatggttgagaaaagtcatccatcttccctccccaccctcccacagcccctcaaccactgccctgaaacttatatgctgttatccgcagctccatctggagcatcacagctactgtcaaccctgacgctctttctgaaaaaacaccggatggacatcagaactatttctttaaggatgttactgagccacacaggaaaacttgccttatgattttgaatgcacggatctgatttgactaaacatgataactagaggatcacccaatctactcccattttcaactctaaatcatcagagtgtctcaaatccaaagcacacacagaccagcctggccaacgcggtgaaactccacccctactaaaagtataaaaattatccaggtgtggtggcgggcgcctgtaatccaagctacttgggagtctgaggcaggagaatcccttgaacctgggagatggaggttgcagtgagcagagatcacaccaccgcactctagcctgggccacaaatcaacaacaacaacaacaacaaaaaacaaagcgcacacagagactgaggtcctctttggcattgagaagatggctatgcaagtcccaactagcaagtgcaaacttcccagcttcacttctgccagtgtcccttcaccccttctcaaccccactgggaggcaggagggtgcttgacaataacagccttggcatcactctgccagggtgtaataggaactgttacaattctgagattctgtgtaagcactggcctttctgcctagaatgccttctcctctcttttttaactgcatgctcctatttatctttcaaagcccggaaaaaataacactgcacacgggaaatgctcccttcctactgcagtcatttagatgactctatgccattccattcatttctctttcctaccacagaagtgctttgagattttggagtcagactgcttgaacttgaatcctggccctctcatcagagacttgacttattttaggcaagttatataaccaattttacctcagttccttacccataaaatgggtctaatgagagtacctaccacacagaattttgatgaaaactgaatgagatgaaggcctttaaggcagtggtccccaaccctggggacacagacaggtaccattttgtggcctgttaggaactgggccacacagcaggaggtgagcagtgggtgagtgagatcagcgttatttacagctgctccccattgctcaccttactgcctgagctccacctcctgtcagatcagcagtggcattaaattctcatagcagcacaaaccctgtcatgaactgcacatgcgagggatctaggttgtgcgctccttatgagaatctaatgcctaatgacctgtcaccgtctcccatcacccctagatgggagtgtctagttgcaggaaacaagctcagggcttccactgattctacattatggtgagttgtataattatttcattatataatacaatgtaataataatagaaacacagtgcacaacaaatgtaatgtgcttgaatcatccccaaaccatcccagtccacggtcttccacattttgtcttttcacaaaattgtcttccacaaaactggtccctggtgccaaaaaggcttgggaccactgctttaaagcctttgcatagtgcttagaattgagggggaaaaaaaaaacaaaaacaatgtagctagttgctacaatcactatattggtgagtttcaaaaggaaaagaattctgtcccatttatgcttgagccttgagttgctaaccaagcctgacacaaaattactgttgaagggatgtgtgagtcctaattgaaatgaggcctcttaagggaattgtggaccaaaccccaagcaggcagaaagccgtatcttaattattgcaagtatttcaggcaaggtgtggatggccatttgaattcaagcagactaggacctgggatgagaaagaaggtgtgtacgtgacttgatctttgaactttagctcaccatctggaagaaggctgagtattctctgcactcacatagtagctaatgcctactccccagccacccacaattctttctgtaggaaggctcgctagaatactttgtgatattggatattagttccatattctactgtgtatcttagttcaaccaaattgtaatcatctgatatttatttcttttaatataaatataagtatattaagtctt

SEQ ID NO: 10 - DNA, 23 bp, Artificial Sequence
  source: /note="Description of Artificial Sequence: Synthetic oligonucleotide"
  misc_feature (1)..(1): /note="5'-Phos"
gttggacttgtacgatagctctc

SEQ ID NO: 11 - DNA, 25 bp, Artificial Sequence
  source: /note="Description of Artificial Sequence: Synthetic oligonucleotide"
  misc_feature (1)..(1): /note="5'-OH"
  modified_base (5)..(5): iBIOdT
  modified_base (20)..(24): a, c, t, g, unknown or other
gctancgtacaagtccaacnnnnnv

SEQ ID NO: 12 - DNA, 19 bp, Artificial Sequence
  source: /note="Description of Artificial Sequence: Synthetic oligonucleotide"
  misc_feature (1)..(1): /note="5'-OH"
gcgatatcactgttccaac

SEQ ID NO: 13 - DNA, 23 bp, Artificial Sequence
  source: /note="Description of Artificial Sequence: Synthetic oligonucleotide"
  misc_feature (1)..(1): /note="5'-OH"
gttggaacagtgatatcgcgaga

SEQ ID NO: 14 - DNA, 21 bp, Artificial Sequence
  source: /note="Description of Artificial Sequence: Synthetic oligonucleotide"
ggccgcgatatcggatccaac

SEQ ID NO: 15 - DNA, 17 bp, Artificial Sequence
  source: /note="Description of Artificial Sequence: Synthetic oligonucleotide"
gttggatccgatatcgc

SEQ ID NO: 16 - DNA, 46 bp, Artificial Sequence
  source: /note="Description of Artificial Sequence: Synthetic oligonucleotide"
  modified_base (45)..(46): a, c, t, g, unknown or other
ccatctcatccctgcgtgtcccatctgttccctccctgtctcagnn

SEQ ID NO: 17 - DNA, 44 bp, Artificial Sequence
  source: /note="Description of Artificial Sequence: Synthetic oligonucleotide"
ctgagacagggagggaacagatgggacacgcagggatgagatgg

SEQ ID NO: 18 - DNA, 44 bp, Artificial Sequence
  source: /note="Description of Artificial Sequence: Synthetic oligonucleotide"
ctgagacacgcaacaggggataggcaaggcacacaggggatagg

SEQ ID NO: 19 - DNA, 46 bp, Artificial Sequence
  source: /note="Description of Artificial Sequence: Synthetic oligonucleotide"
  modified_base (45)..(46): a, c, t, g, unknown or other
cctatcccctgtgtgccttgcctatcccctgttgcgtgtctcagnn

SEQ ID NO: 20 - DNA, 49 bp, Artificial Sequence
  source: /note="Description of Artificial Sequence: Synthetic primer"
aatgatacggcgaccaccgagatctacaccctatcccctgtgtgccttg

SEQ ID NO: 21 - DNA, 48 bp, Artificial Sequence
  source: /note="Description of Artificial Sequence: Synthetic primer"
caagcagaagacggcatacgagatcggtccatctcatccctgcgtgtc

SEQ ID NO: 22 - DNA, 32 bp, Artificial Sequence
  source: /note="Description of Artificial Sequence: Synthetic primer"
gtgccttgcctatcccctgttgcgtgtctcag

SEQ ID NO: 23 - DNA, 32 bp, Artificial Sequence
  source: /note="Description of Artificial Sequence: Synthetic primer"
tgcgtgtcccatctgttccctccctgtctcag